European Patent Specification EP 3 373 950 B1, published May 1, 2024. Title: METHODS AND COMPOSITIONS FOR ASSESSING ANTIBODY SPECIFICITIES. Applicant: SERIMMUNE INC. DAUGHERTY , Patrick KAMATH, Kathy REIFERT, Jack. The sequence listing filed with the application follows.

SEQUENCE LISTING (871 sequences)

SEQ ID NO: 1 - protein, 5 aa, Artificial Sequence
  Synthetic peptide
  MISC_FEATURE (1)..(1): Xaa can be D or E
  misc_feature (3)..(3): Xaa can be any naturally occurring amino acid
  MISC_FEATURE (4)..(4): Xaa can be F, Y or L
XTXXK

SEQ ID NO: 2 - protein, 5 aa, Artificial Sequence
  Synthetic peptide
  misc_feature (3)..(3): Xaa can be any naturally occurring amino acid
DTXFK

SEQ ID NO: 3 - protein, 8 aa, Artificial Sequence
  Synthetic peptide
  misc_feature (2)..(2): Xaa can be any naturally occurring amino acid
  misc_feature (4)..(4): Xaa can be any naturally occurring amino acid
  misc_feature (6)..(7): Xaa can be any naturally occurring amino acid
DXTXFXXK

SEQ ID NO: 4 - protein, 8 aa, Artificial Sequence
  Synthetic peptide
  misc_feature (3)..(4): Xaa can be any naturally occurring amino acid
  misc_feature (7)..(7): Xaa can be any naturally occurring amino acid
  MISC_FEATURE (8)..(8): Xaa can be E or D
QPXXPFXX

SEQ ID NO: 5 - protein, 6 aa, Artificial Sequence
  Synthetic peptide
  misc_feature (3)..(4): Xaa can be any naturally occurring amino acid
QPXXPF

SEQ ID NO: 6 - protein, 8 aa, Artificial Sequence
  Synthetic peptide
  misc_feature (2)..(4): Xaa can be any naturally occurring amino acid
  MISC_FEATURE (7)..(7): Xaa can be P or S
QXXXPFXE

SEQ ID NO: 7 - protein, 5 aa, Artificial Sequence
  Synthetic peptide
PFSEM

SEQ ID NO: 8 - protein, 6 aa, Artificial Sequence
  Synthetic peptide
  misc_feature (5)..(5): Xaa can be any naturally occurring amino acid
  misc_feature (6)..(6): Xaa can be F or W
PFSEXX

SEQ ID NO: 9 - protein, 7 aa, Artificial Sequence
  Synthetic peptide
  misc_feature (4)..(5): Xaa can be any naturally occurring amino acid
  MISC_FEATURE (6)..(6): Xaa can be L or M
LFGXXXN

SEQ ID NO: 10 - protein, 7 aa, Artificial Sequence
  Synthetic peptide
  misc_feature (4)..(5): Xaa can be any naturally occurring amino acid
  MISC_FEATURE (6)..(6): Xaa can be Y or F
EWVXXXD

SEQ ID NO: 11 - protein, 6 aa, Artificial Sequence
  Synthetic peptide
  MISC_FEATURE (2)..(2): Xaa can be L or M
  misc_feature (5)..(5): Xaa can be any naturally occurring amino acid
PXALXL

SEQ ID NO: 12 - protein, 8 aa, Artificial Sequence
  Synthetic peptide
  misc_feature (2)..(2): Xaa can be any naturally occurring amino acid
  misc_feature (5)..(5): Xaa can be any naturally occurring amino acid
  misc_feature (7)..(7): Xaa can be any naturally occurring amino acid
KXNEXWXV

SEQ ID NO: 13 - protein, 7 aa, Artificial Sequence
  Synthetic peptide
  MISC_FEATURE (2)..(2): Xaa can be A or G
  misc_feature (3)..(3): Xaa can be any naturally occurring amino acid
  misc_feature (6)..(6): Xaa can be any naturally occurring amino acid
PXXRTXK

SEQ ID NO: 14 - protein, 6 aa, Artificial Sequence
  Synthetic peptide
  misc_feature (4)..(4): Xaa can be any naturally occurring amino acid
AYTXVN

SEQ ID NO: 15 - protein, 8 aa, Artificial Sequence
  Synthetic peptide
  MISC_FEATURE (3)..(3): Xaa can be A or S
  misc_feature (5)..(7): Xaa can be any naturally occurring amino acid
WNXYXXXN

SEQ ID NO: 16 - protein, 8 aa, Artificial Sequence
  Synthetic peptide
  MISC_FEATURE (1)..(1): Xaa can be R, K or E
  misc_feature (2)..(3): Xaa can be any naturally occurring amino acid
  misc_feature (5)..(5): Xaa can be any naturally occurring amino acid
  MISC_FEATURE (7)..(7): Xaa can be L or M
XXXWXPXQ

SEQ ID NO: 17 - protein, 7 aa, Artificial Sequence
  Synthetic peptide
  MISC_FEATURE (1)..(1): Xaa can be A or S
  misc_feature (3)..(3): Xaa can be any naturally occurring amino acid
  misc_feature (5)..(5): Xaa can be any naturally occurring amino acid
  MISC_FEATURE (6)..(6): Xaa can be S or A
  MISC_FEATURE (7)..(7): Xaa can be Y or F
XYXSXXX

SEQ ID NO: 18 - protein, 7 aa, Artificial Sequence
  Synthetic peptide
  misc_feature (2)..(2): Xaa can be any naturally occurring amino acid
  misc_feature (4)..(4): Xaa can be any naturally occurring amino acid
EXYXSPS

SEQ ID NO: 19 - protein, 6 aa, Artificial Sequence
  Synthetic peptide
  misc_feature (4)..(4): Xaa can be any naturally occurring amino acid
MNIXDD

SEQ ID NO: 20 - protein, 5 aa, Artificial Sequence
  Synthetic peptide
  MISC_FEATURE (3)..(3): Xaa can be A, N or K
EHXFW

SEQ ID NO: 21 - protein, 5 aa, Artificial Sequence
  Synthetic peptide
VHNAY

SEQ ID NO: 22 - protein, 6 aa, Artificial Sequence
  Synthetic peptide
  MISC_FEATURE (3)..(3): Xaa can be E or A
  misc_feature (4)..(4): Xaa can be any naturally occurring amino acid
HGXXLN

SEQ ID NO: 23 - protein, 9 aa, Artificial Sequence
  Synthetic peptide
  MISC_FEATURE (1)..(1): Xaa can be G or D
  misc_feature (2)..(3): Xaa can be any naturally occurring amino acid
  MISC_FEATURE (4)..(4): Xaa can be L or F
  misc_feature (5)..(6): Xaa can be any naturally occurring amino acid
  MISC_FEATURE (8)..(8): Xaa can be M or L
XXXXXXPXQ

SEQ ID NO: 24 - protein, 7 aa, Artificial Sequence
  Synthetic peptide
  MISC_FEATURE (1)..(1): Xaa can be L, V, M or I
  misc_feature (2)..(2): Xaa can be any naturally occurring amino acid
  misc_feature (5)..(5): Xaa can be any naturally occurring amino acid
  MISC_FEATURE (6)..(6): Xaa can be T or S
  MISC_FEATURE (7)..(7): Xaa can be F, G or I
XXNAXXX

SEQ ID NO: 25 - protein, 6 aa, Artificial Sequence
  Synthetic peptide
  misc_feature (2)..(2): Xaa can be any naturally occurring amino acid
PXNSYT

SEQ ID NO: 26 - protein, 9 aa, Artificial Sequence
  Synthetic peptide
  misc_feature (2)..(3): Xaa can be any naturally occurring amino acid
  misc_feature (7)..(8): Xaa can be any naturally occurring amino acid
RXXPLAXXL

SEQ ID NO: 27 - protein, 7 aa, Artificial Sequence
  Synthetic peptide
  misc_feature (4)..(4): Xaa can be any naturally occurring amino acid
  misc_feature (6)..(6): Xaa can be any naturally occurring amino acid
CPKXNXT

SEQ ID NO: 28 - protein, 5 aa, Artificial Sequence
  Synthetic peptide
  MISC_FEATURE (2)..(2): Xaa can be P or A
  MISC_FEATURE (4)..(4): Xaa can be A or M
QXHXF

SEQ ID NO: 29 - protein, 9 aa, Artificial Sequence
  Synthetic peptide
  misc_feature (3)..(3): Xaa can be any naturally occurring amino acid
  misc_feature (6)..(8): Xaa can be any naturally occurring amino acid
  MISC_FEATURE (9)..(9): Xaa can be G, S or P
PAXENXXXX

SEQ ID NO: 30 - protein, 5 aa, Artificial Sequence
  Synthetic peptide
  MISC_FEATURE (4)..(4): Xaa can  be D or E
NIDXD

SEQ ID NO: 31 - protein, 7 aa, Artificial Sequence
  Synthetic peptide
  misc_feature (2)..(2): Xaa can be any naturally occurring amino acid
  misc_feature (4)..(4): Xaa can be any naturally occurring amino acid
  MISC_FEATURE (5)..(5): Xaa can ne V or S
  MISC_FEATURE (5)..(5): Xaa can be V or S
  MISC_FEATURE (7)..(7): Xaa can be N or A
RXQXXDX

SEQ ID NO: 32 - protein, 7 aa, Artificial Sequence
  Synthetic peptide
  misc_feature (2)..(2): Xaa can be any naturally occurring amino acid
  MISC_FEATURE (3)..(3): Xaa can be D or P
  misc_feature (5)..(5): Xaa can be any naturally occurring amino acid
WXXPXHL

SEQ ID NO: 33 - protein, 5 aa, Artificial Sequence
  Synthetic peptide
  MISC_FEATURE (4)..(4): Xaa can be F or I
  MISC_FEATURE (5)..(5): Xaa can be F or I
TWAXX

SEQ ID NO: 34 - protein, 6 aa, Artificial Sequence
  Synthetic peptide
  misc_feature (3)..(3): Xaa can be any naturally occurring amino acid
EDXGHP

SEQ ID NO: 35 - protein, 10 aa, Artificial Sequence
  Synthetic peptide
  MISC_FEATURE (1)..(1): Xaa can be E, T or A
  misc_feature (2)..(4): Xaa can be any naturally occurring amino acid
  MISC_FEATURE (5)..(5): Xaa can be Y or F
  misc_feature (6)..(7): Xaa can be any naturally occurring amino acid
  MISC_FEATURE (9)..(9): Xaa can be S or R
XXXXXXXPXQ

SEQ ID NO: 36 - protein, 6 aa, Artificial Sequence
  Synthetic peptide
  misc_feature (3)..(3): Xaa can be any naturally occurring amino acid
  MISC_FEATURE (5)..(5): Xaa can be R or K
GMXPXQ

SEQ ID NO: 37 - protein, 10 aa, Artificial Sequence
  Synthetic peptide
  misc_feature (2)..(3): Xaa can be any naturally occurring amino acid
  MISC_FEATURE (4)..(4): Xaa can be V or I
  misc_feature (6)..(7): Xaa can be any naturally occurring amino acid
  misc_feature (9)..(9): Xaa can be any naturally occurring amino acid
WXXXRXXPXQ

SEQ ID NO: 38 - protein, 7 aa, Artificial Sequence
  Synthetic peptide
  MISC_FEATURE (1)..(1): Xaa can be N or E
  MISC_FEATURE (2)..(2): Xaa can be A or G
  MISC_FEATURE (4)..(4): Xaa can be S, A or T
  misc_feature (5)..(6): Xaa can be any naturally occurring amino acid
XXYXXXW

SEQ ID NO: 39 - protein, 7 aa, Artificial Sequence
  Synthetic peptide
  misc_feature (2)..(2): Xaa can be any naturally occurring amino acid
  MISC_FEATURE (4)..(4): Xaa can be S or T
  misc_feature (5)..(5): Xaa can be any naturally occurring amino acid
KXIXXYW

SEQ ID NO: 40 - protein, 8 aa, Artificial Sequence
  Synthetic peptide
  misc_feature (3)..(3): Xaa can be any naturally occurring amino acid
  misc_feature (6)..(7): Xaa can be any naturally occurring amino acid
YYXYRXXK

SEQ ID NO: 41 - protein, 7 aa, Artificial Sequence
  Synthetic peptide
  misc_feature (2)..(2): Xaa can be any naturally occurring amino acid
  misc_feature (5)..(5): Xaa can be any naturally occurring amino acid
  MISC_FEATURE (7)..(7): Xaa can  be F or Y
KXHEXGX

SEQ ID NO: 42 - protein, 5 aa, Artificial Sequence
  Synthetic peptide
  MISC_FEATURE (5)..(5): Xaa can be V or I
HHFLX

SEQ ID NO: 43 - protein, 5 aa, Artificial Sequence
  Synthetic peptide
  MISC_FEATURE (1)..(1): Xaa can be L or V
XCNAY

SEQ ID NO: 44 - protein, 7 aa, Artificial Sequence
  Synthetic peptide
LFGANLN

SEQ ID NO: 45 - protein, 7 aa, Artificial Sequence
  Synthetic peptide
PGPRTCK

SEQ ID NO: 46 - protein, 7 aa, Artificial Sequence
  Synthetic peptide
PARRTRK

SEQ ID NO: 47 - protein, 7 aa, Artificial Sequence
  Synthetic peptide
IANAGSI

SEQ ID NO: 48 - protein, 10 aa, Artificial Sequence
  Synthetic peptide
WAQIRHIPYQ

SEQ ID NO: 49 - protein, 6 aa, Artificial Sequence
  Synthetic peptide
MRNPQQ

SEQ ID NO: 50 - protein, 8 aa, Artificial Sequence
  Synthetic peptide
  MISC_FEATURE (2)..(2): Xaa can be E, D or Q
  MISC_FEATURE (5)..(5): Xaa can be L, I or V
  MISC_FEATURE (6)..(6): Xaa can be I or V
  MISC_FEATURE (7)..(7): Xaa can be D or E
LXEVXXXK

SEQ ID NO: 51 - protein, 6 aa, Artificial Sequence
  Synthetic peptide
  MISC_FEATURE (2)..(2): Xaa can be V or I
  MISC_FEATURE (3)..(3): Xaa can be V, I, or L
  MISC_FEATURE (4)..(4): Xaa can be I or V
  MISC_FEATURE (5)..(5): Xaa can be D, E or N
EXXXXK

SEQ ID NO: 52 - protein, 6 aa, Artificial Sequence
  Synthetic peptide
  MISC_FEATURE (2)..(2): Xaa can be V or I
  MISC_FEATURE (3)..(3): Xaa can be V or I
  MISC_FEATURE (4)..(4): Xaa can be V or I
  misc_feature (5)..(5): Xaa can be any naturally occurring amino acid
EXXXXK

SEQ ID NO: 53 - protein, 5 aa, Artificial Sequence
  Synthetic peptide
  misc_feature (2)..(2): Xaa can be any naturally occurring amino acid
VXPNI

SEQ ID NO: 54 - protein, 4 aa, Artificial Sequence
  Synthetic peptide
VVPN

SEQ ID NO: 55 - protein, 9 aa, Artificial Sequence
  Synthetic peptide
  misc_feature (2)..(2): Xaa can be any naturally occurring amino acid
LXEVLVVVP

SEQ ID NO: 56 - protein, 8 aa, Artificial Sequence
  Synthetic peptide
  misc_feature (3)..(3): Xaa can be any naturally occurring amino acid
  misc_feature (6)..(6): Xaa can be any naturally occurring amino acid
GPXHTXKV

SEQ ID NO: 57 - protein, 9 aa, Artificial Sequence
  Synthetic peptide
  misc_feature (2)..(2): Xaa can be any naturally occurring amino acid
  MISC_FEATURE (4)..(4): Xaa can be V or I
  misc_feature (6)..(6): Xaa can be any naturally occurring amino acid
  MISC_FEATURE (7)..(7): Xaa can be V or T
EXYXDXXLN

SEQ ID NO: 58 - protein, 9 aa, Artificial Sequence
  Synthetic peptide
  MISC_FEATURE (6)..(6): Xaa can be I or V
ELEEVXVDK

SEQ ID NO: 59 - protein, 11 aa, Artificial Sequence
  Synthetic peptide
LNEVLVVVPNI

SEQ ID NO: 60 - protein, 8 aa, Artificial Sequence
  Synthetic peptide
GPKHTQKV

SEQ ID NO: 61 - protein, 9 aa, Artificial Sequence
  Synthetic peptide
EEYVDQVLN

SEQ ID NO: 62 - protein, 9 aa, Artificial Sequence
  Synthetic peptide
  misc_feature (2)..(2): Xaa can be any naturally occurring amino acid
  misc_feature (6)..(7): Xaa can be any naturally occurring amino acid
  MISC_FEATURE (9)..(9): Xaa can be S or T
KXDPDXXWX

SEQ ID NO: 63 - protein, 7 aa, Artificial Sequence
  Synthetic peptide
  misc_feature (3)..(3): Xaa can be any naturally occurring amino acid
KPXLGGK

SEQ ID NO: 64 - protein, 9 aa, Artificial Sequence
  Synthetic peptide
  misc_feature (2)..(2): Xaa can be any naturally occurring amino acid
  misc_feature (6)..(7): Xaa can be any naturally occurring amino acid
KXDPDXXWT

SEQ ID NO: 65 - protein, 7 aa, Artificial Sequence
  Synthetic peptide
KPTLGGK

SEQ ID NO: 66 - protein, 8 aa, Artificial Sequence
  Synthetic peptide
  MISC_FEATURE (1)..(1): Xaa can be I or V
  misc_feature (2)..(2): Xaa can be any naturally occurring amino acid
  MISC_FEATURE (3)..(3): Xaa can be P or R
XXXQPEKP

SEQ ID NO: 67 - protein, 7 aa, Artificial Sequence
  Synthetic peptide
  misc_feature (2)..(2): Xaa can be any naturally occurring amino acid
KXDDMLN

SEQ ID NO: 68 - protein, 7 aa, Artificial Sequence
  Synthetic peptide
  misc_feature (2)..(2): Xaa can be any naturally occurring amino acid
  misc_feature (4)..(4): Xaa can be any naturally occurring amino acid
KXDXMLN

SEQ ID NO: 69 - protein, 9 aa, Artificial Sequence
  Synthetic peptide
  MISC_FEATURE (1)..(1): Xaa can be L or W
  misc_feature (2)..(2): Xaa can be any naturally occurring amino acid
  misc_feature (6)..(6): Xaa can be any naturally occurring amino acid
XXSAEXEEK

SEQ ID NO: 70 - protein, 7 aa, Artificial Sequence
  Synthetic peptide
  misc_feature (4)..(4): Xaa can be any naturally occurring amino acid
  misc_feature (6)..(6): Xaa can be any naturally occurring amino acid
SAEXEXK

SEQ ID NO: 71 - protein, 8 aa, Artificial Sequence
  Synthetic peptide
VKPQPEKP

SEQ ID NO: 72 - protein, 7 aa, Artificial Sequence
  Synthetic peptide
KTDDMLN

SEQ ID NO: 73 - protein, 9 aa, Artificial Sequence
  Synthetic peptide
LESAEKEEK

SEQ ID NO: 74 - protein, 6 aa, Artificial Sequence
  Synthetic peptide
  misc_feature (3)..(3): Xaa can be any naturally occurring amino acid
  MISC_FEATURE (5)..(5): Xaa can be F or Y
HEXEXQ

SEQ ID NO: 75 - protein, 6 aa, Artificial Sequence
  Synthetic peptide
  MISC_FEATURE (3)..(3): Xaa can be M, L or F
  misc_feature (5)..(5): Xaa can be any naturally occurring amino acid
LDXWXE

SEQ ID NO: 76 - protein, 5 aa, Artificial Sequence
  Synthetic peptide
HCSAC

SEQ ID NO: 77 - protein, 6 aa, Artificial Sequence
  Synthetic peptide
  MISC_FEATURE (1)..(1): Xaa can be F or Y
  misc_feature (2)..(2): Xaa can be any naturally occurring amino acid
XXGVVN

SEQ ID NO: 78 - protein, 9 aa, Artificial Sequence
  Synthetic peptide
  misc_feature (2)..(4): Xaa can be any naturally occurring amino acid
  misc_feature (8)..(8): Xaa can be any naturally occurring amino acid
KXXXGRGXI

SEQ ID NO: 79 - protein, 5 aa, Artificial Sequence
  Synthetic peptide
  MISC_FEATURE (4)..(4): Xaa can be L or A
GPHXE

SEQ ID NO: 80 - protein, 5 aa, Artificial Sequence
  Synthetic peptide
PRREP

SEQ ID NO: 81 - protein, 8 aa, Artificial Sequence
  Synthetic peptide
  misc_feature (3)..(5): Xaa can be any naturally occurring amino acid
CNXXXECY

SEQ ID NO: 82 - protein, 8 aa, Artificial Sequence
  Synthetic peptide
  misc_feature (2)..(2): Xaa can be any naturally occurring amino acid
  misc_feature (6)..(7): Xaa can be any naturally occurring amino acid
KXCQPXXC

SEQ ID NO: 83 - protein, 6 aa, Artificial Sequence
  Synthetic peptide
  misc_feature (2)..(2): Xaa can be any naturally occurring amino acid
  MISC_FEATURE (5)..(5): Xaa can be F or H
  MISC_FEATURE (6)..(6): Xaa can be T or S
PXPDXX

SEQ ID NO: 84 - protein, 10 aa, Artificial Sequence
  Synthetic peptide
  misc_feature (2)..(4): Xaa can be any naturally occurring amino acid
  misc_feature (6)..(6): Xaa can be any naturally occurring amino acid
  MISC_FEATURE (8)..(8): Xaa can be A or G
  misc_feature (9)..(9): Xaa can be any naturally occurring amino acid
NXXXEXYXXD

SEQ ID NO: 85 - protein, 7 aa, Artificial Sequence
  Synthetic peptide
  MISC_FEATURE (2)..(2): Xaa can be A or G
  misc_feature (4)..(5): Xaa can be any naturally occurring amino acid
PXAXXLD

SEQ ID NO: 86 - protein, 7 aa, Artificial Sequence
  Synthetic peptide
  misc_feature (4)..(4): Xaa can be any naturally occurring amino acid
  misc_feature (6)..(6): Xaa can be any naturally occurring amino acid
MPSXSXE

SEQ ID NO: 87 - protein, 7 aa, Artificial Sequence
  Synthetic peptide
  MISC_FEATURE (1)..(1): Xaa can be R or K
  misc_feature (2)..(2): Xaa can be any naturally occurring amino acid
  misc_feature (4)..(4): Xaa can be any naturally occurring amino acid
  MISC_FEATURE (7)..(7): Xaa can be T or S
XXYXHRX

SEQ ID NO: 88 - protein, 8 aa, Artificial Sequence
  Synthetic peptide
  MISC_FEATURE (2)..(2): Xaa can be P or A
  misc_feature (3)..(3): Xaa can be any naturally occurring amino acid
  misc_feature (5)..(5): Xaa can be any naturally occurring amino acid
  misc_feature (7)..(7): Xaa can be any naturally occurring amino acid
KXXFXFXK

SEQ ID NO: 89 - protein, 7 aa, Artificial Sequence
  Synthetic peptide
  MISC_FEATURE (3)..(3): Xaa can be C, S or T
  misc_feature (4)..(4): Xaa can be any naturally occurring amino acid
  misc_feature (6)..(6): Xaa can be any naturally occurring amino acid
DDXXGXR

SEQ ID NO: 90 - protein, 8 aa, Artificial Sequence
  Synthetic peptide
  MISC_FEATURE (2)..(2): Xaa can be M or L
  misc_feature (3)..(4): Xaa can be any naturally occurring amino acid
  misc_feature (6)..(6): Xaa can be any naturally occurring amino acid
PXXXHXMY

SEQ ID NO: 91 - protein, 7 aa, Artificial Sequence
  Synthetic peptide
  misc_feature (2)..(2): Xaa can be any naturally occurring amino acid
  MISC_FEATURE (3)..(3): Xaa can be A, S or Q
  MISC_FEATURE (4)..(4): Xaa can be S, A or T
  misc_feature (5)..(5): Xaa can be any naturally occurring amino acid
KXXXXRG

SEQ ID NO: 92 - protein, 5 aa, Artificial Sequence
  Synthetic peptide
  MISC_FEATURE (1)..(1): Xaa can be D or G
XQPEN

SEQ ID NO: 93 - protein, 5 aa, Artificial Sequence
  Synthetic peptide
  MISC_FEATURE (1)..(1): Xaa can be K, H or R
  MISC_FEATURE (3)..(3): Xaa can be Q or N
XNXDG

SEQ ID NO: 94 - protein, 7 aa, Artificial Sequence
  Synthetic peptide
  misc_feature (2)..(2): Xaa can be any naturally occurring amino acid
  MISC_FEATURE (3)..(3): Xaa can be E, V or S
  misc_feature (6)..(6): Xaa can be any naturally occurring amino acid
NXXGEXY

SEQ ID NO: 95 - protein, 5 aa, Artificial Sequence
  Synthetic peptide
  MISC_FEATURE (3)..(3): Xaa can be V or I
EPXTG

SEQ ID NO: 96 - protein, 5 aa, Artificial Sequence
  Synthetic peptide
  MISC_FEATURE (4)..(4): Xaa can be P or A
  MISC_FEATURE (5)..(5): Xaa can be K or R
HGMXX

SEQ ID NO: 97 - protein, 5 aa, Artificial Sequence
  Synthetic peptide
  MISC_FEATURE (1)..(1): Xaa can be V, I or T
XPWIF

SEQ ID NO: 98 - protein, 7 aa, Artificial Sequence
  Synthetic peptide
  misc_feature (2)..(2): Xaa can be any naturally occurring amino acid
  MISC_FEATURE (3)..(3): Xaa can be S, T or N
  misc_feature (5)..(5): Xaa can be any naturally occurring amino acid
KXXVXFQ

SEQ ID NO: 99 - protein, 5 aa, Artificial Sequence
  Synthetic peptide
  MISC_FEATURE: Xaa can be V, A or I
  MISC_FEATURE (1)..(1): Xaa can be V, A or I
XWSGS

SEQ ID NO: 100 - protein, 7 aa, Artificial Sequence
  Synthetic peptide
  MISC_FEATURE (3)..(3): Xaa can be L, I, A or M
  misc_feature (4)..(5): Xaa can be any naturally occurring amino acid
FSXXXWG

SEQ ID NO: 101 - protein, 5 aa, Artificial Sequence
  Synthetic peptide
  MISC_FEATURE (4)..(4): Xaa can be P or Q
PTNXG

SEQ ID NO: 102 - protein, 9 aa, Artificial Sequence
  Synthetic peptide
  MISC_FEATURE (1)..(1): Xaa can be R or K
  misc_feature (3)..(4): Xaa can be any naturally occurring amino acid
  MISC_FEATURE (5)..(5): Xaa can be Y or W
  misc_feature (6)..(6): Xaa can be any naturally occurring amino acid
  misc_feature (8)..(8): Xaa can be any naturally occurring amino acid
  MISC_FEATURE (9)..(9): Xaa can be T or S
XKXXXXHXX

SEQ ID NO: 103 - protein, 7 aa, Artificial Sequence
  Synthetic peptide
  MISC_FEATURE (1)..(1): Xaa can be H, R or W
  misc_feature (2)..(3): Xaa can be any naturally occurring amino acid
XXXHPRF

SEQ ID NO: 104 - protein, 6 aa, Artificial Sequence
  Synthetic peptide
  MISC_FEATURE (1)..(1): Xaa can be R or K
  misc_feature (4)..(4): Xaa can be any naturally occurring amino acid
XMRXID

SEQ ID NO: 105 - protein, 6 aa, Artificial Sequence
  Synthetic peptide
  misc_feature (3)..(3): Xaa can be any naturally occurring amino acid
QHXGHP

SEQ ID NO: 106 - protein, 7 aa, Artificial Sequence
  Synthetic peptide
  misc_feature (2)..(3): Xaa can be any naturally occurring amino acid
KXXLPED

SEQ ID NO: 107 - protein, 7 aa, Artificial Sequence
  Synthetic peptide
  MISC_FEATURE (1)..(1): Xaa can be I or V
  misc_feature (3)..(4): Xaa can be any naturally occurring amino acid
XLXXFGY

SEQ ID NO: 108 - protein, 9 aa, Artificial Sequence
  Synthetic peptide
  misc_feature (4)..(7): Xaa can be any naturally occurring amino acid
PLDXXXXIS

SEQ ID NO: 109 - protein, 7 aa, Artificial Sequence
  Synthetic peptide
  misc_feature (3)..(3): Xaa can be any naturally occurring amino acid
  misc_feature (6)..(6): Xaa can be any naturally occurring amino acid
ETXIPXE

SEQ ID NO: 110 - protein, 8 aa, Artificial Sequence
  Synthetic peptide
  MISC_FEATURE (1)..(1): Xaa can be V or I
  misc_feature (3)..(3): Xaa can be any naturally occurring amino acid
  MISC_FEATURE (4)..(4): Xaa can be D or E
  MISC_FEATURE (5)..(5): Xaa can be M or L
  misc_feature (7)..(7): Xaa can be any naturally occurring amino acid
XNXXXYXP

SEQ ID NO: 111 - protein, 7 aa, Artificial Sequence
  Synthetic peptide
  misc_feature (3)..(4): Xaa can be any naturally occurring amino acid
FLXXIGA

SEQ ID NO: 112 - protein, 7 aa, Artificial Sequence
  Synthetic peptide
  MISC_FEATURE (2)..(2): Xaa can be V or I
  misc_feature (3)..(3): Xaa can be any naturally occurring amino acid
  MISC_FEATURE (4)..(4): Xaa can be M or I
  MISC_FEATURE (5)..(5): Xaa can be I, L or V
  misc_feature (6)..(6): Xaa can be any naturally occurring amino acid
  MISC_FEATURE (7)..(7): Xaa can be K or R
  MISC_FEATURE (7)..(7)
DXXXXXX

SEQ ID NO: 113 - protein, 8 aa, Artificial Sequence
  Synthetic peptide
  misc_feature (2)..(2): Xaa can be any naturally occurring amino acid
  misc_feature (6)..(6): Xaa can be any naturally occurring amino acid
  MISC_FEATURE (7)..(7): Xaa can be I or L
RXSPYXXF

SEQ ID NO: 114 - protein, 5 aa, Artificial Sequence
  Synthetic peptide
VGPRH

SEQ ID NO: 115 - protein, 6 aa, Artificial Sequence
  Synthetic peptide
  misc_feature (3)..(3): Xaa can be any naturally occurring amino acid
  MISC_FEATURE (6)..(6): Xaa can be E or D
PQXQHX

SEQ ID NO: 116 - protein, 7 aa, Artificial Sequence
  Synthetic peptide
  misc_feature (2)..(3): Xaa can be any naturally occurring amino acid
PXXGGFG

SEQ ID NO: 117 - protein, 8 aa, Artificial Sequence
  Synthetic peptide
  misc_feature (2)..(2): Xaa can be any naturally occurring amino acid
  misc_feature (5)..(6): Xaa can be any naturally occurring amino acid
KXEGXXMG

SEQ ID NO: 118 - protein, 10 aa, Artificial Sequence
  Synthetic peptide
  misc_feature (2)..(3): Xaa can be any naturally occurring amino acid
  misc_feature (5)..(5): Xaa can be any naturally occurring amino acid
  misc_feature (7)..(8): Xaa can be any naturally occurring amino acid
KXXGXTXXLS

SEQ ID NO: 119 - protein, 5 aa, Artificial Sequence
  Synthetic peptide
  MISC_FEATURE (4)..(4): Xaa can be F or W
EMGXQ

SEQ ID NO: 120 - protein, 9 aa, Artificial Sequence
  Synthetic peptide
  MISC_FEATURE (1)..(1): Xaa can be V or I
  misc_feature (3)..(3): Xaa can be any naturally occurring amino acid
  misc_feature (5)..(6): Xaa can be any naturally occurring amino acid
  misc_feature (8)..(8): Xaa can be any naturally occurring amino acid
XKXGXXDXP

SEQ ID NO: 121 - protein, 7 aa, Artificial Sequence
  Synthetic peptide
  MISC_FEATURE (3)..(3): Xaa can be D or N
  misc_feature (5)..(5): Xaa can be any naturally occurring amino acid
PEXEXYP

SEQ ID NO: 122 - protein, 5 aa, Artificial Sequence
  Synthetic peptide
HYEWA

SEQ ID NO: 123 - protein, 6 aa, Artificial Sequence
  Synthetic peptide
  MISC_FEATURE (1)..(1): Xaa can be H or R
  misc_feature (5)..(5): Xaa can be any naturally occurring amino acid
XSNMXF

SEQ ID NO: 124 - protein, 7 aa, Artificial Sequence
  Synthetic peptide
  MISC_FEATURE (2)..(2): Xaa can be T or V
  misc_feature (4)..(5): Xaa can be any naturally occurring amino acid
MXGXXYE

SEQ ID NO: 125 - protein, 9 aa, Artificial Sequence
  Synthetic peptide
  misc_feature (2)..(3): Xaa can be any naturally occurring amino acid
  MISC_FEATURE (4)..(4): Xaa can be K or H
  misc_feature (6)..(7): Xaa can be any naturally occurring amino acid
DXXXEXXLL

SEQ ID NO: 126 - protein, 9 aa, Artificial Sequence
  Synthetic peptide
  misc_feature (2)..(3): Xaa can be any naturally occurring amino acid
  misc_feature (5)..(5): Xaa can be any naturally occurring amino acid
  MISC_FEATURE (6)..(6): Xaa can be E, D or A
  misc_feature (7)..(7): Xaa can be any naturally occurring amino acid
  MISC_FEATURE (8)..(8): Xaa can be I or V
  MISC_FEATURE (9)..(9): Xaa can be A or R
RXXWXXXXX

SEQ ID NO: 127 - protein, 9 aa, Artificial Sequence
  Synthetic peptide
  misc_feature (2)..(2): Xaa can be any naturally occurring amino acid
  misc_feature (4)..(5): Xaa can be any naturally occurring amino acid
  misc_feature (7)..(7): Xaa can be any naturally occurring amino acid
  MISC_FEATURE (8)..(8): Xaa can be G, P or A
  MISC_FEATURE (9)..(9): Xaa can be T or S
PXDXXAXXX

SEQ ID NO: 128 - protein, 8 aa, Artificial Sequence
  Synthetic peptide
  misc_feature (3)..(4): Xaa can be any naturally occurring amino acid
  misc_feature (6)..(6): Xaa can be any naturally occurring amino acid
  MISC_FEATURE (8)..(8): Xaa can be A, R or G
PDXXSXTX

SEQ ID NO: 129 - protein, 6 aa, Artificial Sequence
  Synthetic peptide
  misc_feature (4)..(4): Xaa can be any naturally occurring amino acid
GREXDG

SEQ ID NO: 130 - protein, 8 aa, Artificial Sequence
  Synthetic peptide
  misc_feature (5)..(7): Xaa can be any naturally occurring amino acid
GVPGXXXK

SEQ ID NO: 131 - protein, 10 aa, Artificial Sequence
  Synthetic peptide
  MISC_FEATURE (1)..(1): Xaa can be L or M
  misc_feature (2)..(4): Xaa can be any naturally occurring amino acid
  MISC_FEATURE (5)..(5): Xaa can be E, D or Q
  misc_feature (7)..(8): Xaa can be any naturally occurring amino acid
XXXXXVXXIM

SEQ ID NO: 132 - protein, 8 aa, Artificial Sequence
  Synthetic peptide
  misc_feature (2)..(4): Xaa can be any naturally occurring amino acid
SXXXVSGG

SEQ ID NO: 133 - protein, 6 aa, Artificial Sequence
  Synthetic peptide
  MISC_FEATURE (2)..(2): Xaa can be K or R
  MISC_FEATURE (5)..(5): Xaa can be D or N
AXAGXK

SEQ ID NO: 134 - protein, 6 aa, Artificial Sequence
  Synthetic peptide
  MISC_FEATURE (2)..(2): Xaa can be R or N
  misc_feature (3)..(3): Xaa can be any naturally occurring amino acid
  MISC_FEATURE (6)..(6): Xaa can be R or Q
FXXINX

SEQ ID NO: 135 - protein, 9 aa, Artificial Sequence
  Synthetic peptide
  misc_feature (2)..(2): Xaa can be any naturally occurring amino acid
  misc_feature (5)..(5): Xaa can be any naturally occurring amino acid
  misc_feature (7)..(7): Xaa can be any naturally occurring amino acid
YXPVXPXSY

SEQ ID NO: 136 - protein, 6 aa, Artificial Sequence
  Synethetic peptide
  misc_feature (2)..(2): Xaa can be any naturally occurring amino acid
KXTFPD

SEQ ID NO: 137 - protein, 7 aa, Artificial Sequence
  Synethetic peptide
  MISC_FEATURE (4)..(4): Xaa can be F, V or M
  misc_feature (5)..(6): Xaa can be any naturally occurring amino acid
PFMXXXR

SEQ ID NO: 138 - protein, 5 aa, Artificial Sequence
  Synethetic peptide
EFWEP

SEQ ID NO: 139 - protein, 5 aa, Artificial Sequence
  Synethetic peptide
  MISC_FEATURE (1)..(1): Xaa can be F or Y
XGALS

SEQ ID NO: 140 - protein, 6 aa, Artificial Sequence
  Synethetic peptide
  misc_feature (2)..(2): Xaa can be any naturally occurring amino acid
PXGTEN

SEQ ID NO: 141 - protein, 6 aa, Artificial Sequence
  Synthetic peptide
  misc_feature (2)..(2): Xaa can be any naturally occurring amino acid
  MISC_FEATURE (3)..(3): Xaa can be K or E
GXXPWE

SEQ ID NO: 142 - protein, 6 aa, Artificial Sequence
  Synthetic peptide
  MISC_FEATURE (2)..(2): Xaa can be I or V
  misc_feature (4)..(4): Xaa can be any naturally occurring amino acid
  MISC_FEATURE (5)..(5): Xaa can be Y or F
  MISC_FEATURE (6)..(6): Xaa can be W or N
DXTXXX

SEQ ID NO: 143 - protein, 6 aa, Artificial Sequence
  Synthetic peptide
QHKGHP

SEQ ID NO: 144 - protein, 6 aa, Artificial Sequence
  Synthetic peptide
QHIGHP

SEQ ID NO: 145 - protein, 7 aa, Artificial Sequence
  Synthetic peptide
KALLPED

SEQ ID NO: 146 - protein, 7 aa, Artificial Sequence
  Synthetic peptide
KKHLPED

SEQ ID NO: 147 - protein, 7 aa, Artificial Sequence
  Synthetic peptide
KITLPED

SEQ ID NO: 148 - protein, 7 aa, Artificial Sequence
  Synthetic peptide
KTILPED

SEQ ID NO: 149 - protein, 7 aa, Artificial Sequence
  Synthetic peptide
KVLLPED

SEQ ID NO: 150 - protein, 7 aa, Artificial Sequence
  Synthetic peptide
VLKKFGY

SEQ ID NO: 151 - protein, 6 aa, Artificial Sequence
  Synthetic peptide
LHLFGY

SEQ ID NO: 152 - protein, 7 aa, Artificial Sequence
  Synthetic peptide
VLGEFGY

SEQ ID NO: 153 - protein, 7 aa, Artificial Sequence
  Synthetic peptide
VLEPFGY

SEQ ID NO: 154 - protein, 9 aa, Artificial Sequence
  Synthetic peptide
PLDVEKEIS

SEQ ID NO: 155 - protein, 9 aa, Artificial Sequence
  Synthetic peptide
PLDLLKYIS

SEQ ID NO: 156 - protein, 7 aa, Artificial Sequence
  Synthetic peptide
ETKIPSE

SEQ ID NO: 157 - protein, 7 aa, Artificial Sequence
  Synthetic peptide
ETEIPSE

SEQ ID NO: 158 - protein, 7 aa, Artificial Sequence
  Synthetic peptide
ETGIPFE

SEQ ID NO: 159 - protein, 8 aa, Artificial Sequence
  Synthetic peptide
VNVDLYIP

SEQ ID NO: 160 - protein, 7 aa, Artificial Sequence
  Synthetic peptide
FLGAIGA

SEQ ID NO: 161 - protein, 7 aa, Artificial Sequence
  Synthetic peptide
FLLFIGA

SEQ ID NO: 162 - protein, 7 aa, Artificial Sequence
  Synthetic peptide
FLKAIGA

SEQ ID NO: 163 - protein, 7 aa, Artificial Sequence
  Synthetic peptide
DIKMIER

SEQ ID NO: 164 - protein, 7 aa, Artificial Sequence
  Synthetic peptide
DIIIVSR

SEQ ID NO: 165 - protein, 7 aa, Artificial Sequence
  Synthetic peptide
DVHMLVR

SEQ ID NO: 166 - protein, 7 aa, Artificial Sequence
  Synthetic peptide
DVDILER

SEQ ID NO: 167 - protein, 8 aa, Artificial Sequence
  Synthetic peptide
RVSPYSIF

SEQ ID NO: 168 - protein, 5 aa, Artificial Sequence
  Synthetic peptide
VGPRH

SEQ ID NO: 169 - protein, 6 aa, Artificial Sequence
  Synthetic peptide
PQKQHE

SEQ ID NO: 170 - protein, 6 aa, Artificial Sequence
  Synthetic peptide
PQGQHD

SEQ ID NO: 171 - protein, 8 aa, Artificial Sequence
  Synthetic peptide
KSEGEFMG

SEQ ID NO: 172 - protein, 8 aa, Artificial Sequence
  Synthetic peptide
KDEGLAMG

SEQ ID NO: 173 - protein, 10 aa, Artificial Sequence
  Synthetic peptide
KDNGSTWSLS

SEQ ID NO: 174 - protein, 10 aa, Artificial Sequence
  Synthetic peptide
KDDGSTWALS

SEQ ID NO: 175 - protein, 9 aa, Artificial Sequence
  Synthetic peptide
IKQGRLDRP

SEQ ID NO: 176 - protein, 5 aa, Artificial Sequence
  Synthetic peptide
HYEWA

SEQ ID NO: 177 - protein, 7 aa, Artificial Sequence
  Synthetic peptide
MVGEHYE

SEQ ID NO: 178 - protein, 7 aa, Artificial Sequence
  Synthetic peptide
MVGKAYE

SEQ ID NO: 179 - protein, 9 aa, Artificial Sequence
  Synthetic peptide
DQLKEGRLL

SEQ ID NO: 180 - protein, 9 aa, Artificial Sequence
  Synthetic peptide
DVVKELMLL

SEQ ID NO: 181 - protein, 9 aa, Artificial Sequence
  Synthetic peptide
DLEKENELL

SEQ ID NO: 182 - protein, 9 aa, Artificial Sequence
  Synthetic peptide
DLDKEVSLL

SEQ ID NO: 183 - protein, 9 aa, Artificial Sequence
  Synthetic peptide
RHQWYAVVA

SEQ ID NO: 184 - protein, 9 aa, Artificial Sequence
  Synthetic peptide
RHSWFDDVR

SEQ ID NO: 185 - protein, 9 aa, Artificial Sequence
  Synthetic peptide
RKEWYDVVA

SEQ ID NO: 186 - protein, 9 aa, Artificial Sequence
  Synthetic peptide
RDRWTESIA

SEQ ID NO: 187 - protein, 9 aa, Artificial Sequence
  Synthetic peptide
RATWLDQVR

SEQ ID NO: 188 - protein, 9 aa, Artificial Sequence
  Synthetic peptide
RYVWNEWVA

SEQ ID NO: 189 - protein, 9 aa, Artificial Sequence
  Synthetic peptide
PVDSTAHGT

SEQ ID NO: 190 - protein, 9 aa, Artificial Sequence
  Synthetic peptide
PLDCPALGS

SEQ ID NO: 191 - protein, 9 aa, Artificial Sequence
  Synthetic peptide
PADSSAHGT

SEQ ID NO: 192 - protein, 9 aa, Artificial Sequence
  Synthetic peptide
PKDVKATGS

SEQ ID NO: 193 - protein, 8 aa, Artificial Sequence
  Synthetic peptide
PDVSASGT

SEQ ID NO: 194 - protein, 9 aa, Artificial Sequence
  Synthetic peptide
PGDLPAKAT

SEQ ID NO: 195 - protein, 9 aa, Artificial Sequence
  Synthetic peptide
PADVSAQAT

SEQ ID NO: 196 - protein, 9 aa, Artificial Sequence
  Synthetic peptide
PPDVPASGT

SEQ ID NO: 197 - protein, 8 aa, Artificial Sequence
  Synthetic peptide
PDPASITA

SEQ ID NO: 198 - protein, 8 aa, Artificial Sequence
  Synthetic peptide
PDASSSTA

SEQ ID NO: 199 - protein, 8 aa, Artificial Sequence
  Synthetic peptide
PDSRSITA

SEQ ID NO: 200 - protein, 8 aa, Artificial Sequence
  Synthetic peptide
PDSRSVTA

SEQ ID NO: 201 - protein, 8 aa, Artificial Sequence
  Synthetic peptide
PDSKSPTA

SEQ ID NO: 202 - protein, 8 aa, Artificial Sequence
  Synthetic peptide
PDSESPTA

SEQ ID NO: 203 - protein, 6 aa, Artificial Sequence
  Synthetic peptide
GRESDG

SEQ ID NO: 204 - protein, 6 aa, Artificial Sequence
  Synthetic peptide
GREADG

SEQ ID NO: 205 - protein, 8 aa, Artificial Sequence
  Synthetic peptide
GVPGSHAK

SEQ ID NO: 206 - protein, 8 aa, Artificial Sequence
  Synthetic peptide
GVPGCVIK

SEQ ID NO: 207 - protein, 10 aa, Artificial Sequence
  Synthetic peptide
LSPREVYTIM

SEQ ID NO: 208 - protein, 10 aa, Artificial Sequence
  Synthetic peptide
LTNTDVTRIM

SEQ ID NO: 209 - protein, 10 aa, Artificial Sequence
  Synthetic peptide
LEDEDVLQIM

SEQ ID NO: 210 - protein, 10 aa, Artificial Sequence
  Synthetic peptide
MADPEVAAIM

SEQ ID NO: 211 - protein, 8 aa, Artificial Sequence
  Synthetic peptide
SQADVSGG

SEQ ID NO: 212 - protein, 8 aa, Artificial Sequence
  Synthetic peptide
SVGSVSGG

SEQ ID NO: 213 - protein, 8 aa, Artificial Sequence
  Synthetic peptide
SPSGVSGG

SEQ ID NO: 214 - protein, 8 aa, Artificial Sequence
  Synthetic peptide
SWFDVSGG

SEQ ID NO: 215 - protein, 6 aa, Artificial Sequence
  Synthetic peptide
FRIINQ

SEQ ID NO: 216 - protein, 6 aa, Artificial Sequence
  Synthetic peptide
FRAINR

SEQ ID NO: 217 - protein, 6 aa, Artificial Sequence
  Synthetic peptide
KQTFPD

SEQ ID NO: 218 - protein, 6 aa, Artificial Sequence
  Synthetic peptide
KATFPD

SEQ ID NO: 219 - protein, 7 aa, Artificial Sequence
  Synthetic peptide
PFMVQMR

SEQ ID NO: 220 - protein, 5 aa, Artificial Sequence
  Synthetic peptide
FGALS

SEQ ID NO: 221 - protein, 5 aa, Artificial Sequence
  Synthetic peptide
YGALS

SEQ ID NO: 222 - protein, 6 aa, Artificial Sequence
  Synthetic peptide
PSGTEN

SEQ ID NO: 223 - protein, 6 aa, Artificial Sequence
  Synthetic peptide
GFKPWE

SEQ ID NO: 224 - protein, 6 aa, Artificial Sequence
  Synthetic peptide
DITDYN

SEQ ID NO: 225 - protein, 6 aa, Artificial Sequence
  Synthetic peptide
DVTGFN

SEQ ID NO: 226 - protein, 6 aa, Artificial Sequence
  Synthetic peptide
  misc_feature (2)..(2): Xaa can be any naturally occurring amino acid
  MISC_FEATURE (6)..(6): Xaa can be Q, E or A
AXSPNX

SEQ ID NO: 227 - protein, 9 aa, Artificial Sequence
  Synthetic peptide
  MISC_FEATURE (1)..(1): Xaa can be R or P
  misc_feature (2)..(2): Xaa can be any naturally occurring amino acid
  misc_feature (4)..(4): Xaa can be any naturally occurring amino acid
  misc_feature (6)..(6): Xaa can be any naturally occurring amino acid
  misc_feature (8)..(8): Xaa can be any naturally occurring amino acid
  MISC_FEATURE (9)..(9): Xaa can be I, F, M, L or V
XXAXSXNXX

SEQ ID NO: 228 - protein, 7 aa, Artificial Sequence
  Synthetic peptide
  misc_feature (2)..(3): Xaa can be any naturally occurring amino acid
  MISC_FEATURE (7)..(7): Xaa can be V or T
NXXLGLX

SEQ ID NO: 229 - protein, 8 aa, Artificial Sequence
  Synthetic peptide
  MISC_FEATURE (1)..(1): Xaa can be Y or F
  misc_feature (2)..(2): Xaa can be any naturally occurring amino acid
  MISC_FEATURE (3)..(3): Xaa can be D or E
  misc_feature (5)..(6): Xaa can be any naturally occurring amino acid
XXXIXXFF

SEQ ID NO: 230 - protein, 7 aa, Artificial Sequence
  Synthetic peptide
  misc_feature (2)..(2): Xaa can be any naturally occurring amino acid
  misc_feature (6)..(6): Xaa can be any naturally occurring amino acid
IXHFFXG

SEQ ID NO: 231 - protein, 7 aa, Artificial Sequence
  Synthetic peptide
  MISC_FEATURE (1)..(1): Xaa can be I, L or M
  MISC_FEATURE (2)..(2): Xaa can be I, L or M
  MISC_FEATURE (3)..(3): Xaa can be R or K
  MISC_FEATURE (5)..(5): Xaa can be E or D
  misc_feature (6)..(6): Xaa can be any naturally occurring amino acid
XXXHXXQ

SEQ ID NO: 232 - protein, 6 aa, Artificial Sequence
  Synthetic peptide
  MISC_FEATURE (1)..(1): Xaa can be I, L or M
  MISC_FEATURE (2)..(2): Xaa can be R or K
  misc_feature (5)..(5): Xaa can be any naturally occurring amino acid
XXHEXQ

SEQ ID NO: 233 - protein, 9 aa, Artificial Sequence
  Synthetic peptide
  misc_feature (3)..(4): Xaa can be any naturally occurring amino acid
  MISC_FEATURE (5)..(5): Xaa can be I or L
  misc_feature (6)..(6): Xaa can be any naturally occurring amino acid
  misc_feature (8)..(8): Xaa can be any naturally occurring amino acid
  MISC_FEATURE (9)..(9): Xaa can be K or R
KPXXXXLXX

SEQ ID NO: 234 - protein, 10 aa, Artificial Sequence
  Synthetic peptide
  misc_feature (2)..(2): Xaa can be any naturally occurring amino acid
  misc_feature (4)..(5): Xaa can be any naturally occurring amino acid
  misc_feature (8)..(9): Xaa can be any naturally occurring amino acid
  MISC_FEATURE (10)..(10): Xaa can be W or F
NXDXXYYXXX

SEQ ID NO: 235 - protein, 5 aa, Artificial Sequence
  Synthetic peptide
GLDGP

SEQ ID NO: 236 - protein, 8 aa, Artificial Sequence
  Synthetic peptide
  misc_feature (3)..(3): Xaa can be any naturally occurring amino acid
  misc_feature (6)..(7): Xaa can be any naturally occurring amino acid
RSXHDXXN

SEQ ID NO: 237 - protein, 6 aa, Artificial Sequence
  Synthetic peptide
  misc_feature (3)..(3): Xaa can be any naturally occurring amino acid
  MISC_FEATURE (6)..(6): Xaa can be I or L
FDXFNX

SEQ ID NO: 238 - protein, 6 aa, Artificial Sequence
  Synthetic peptide
  misc_feature (4)..(4): Xaa can be any naturally occurring amino acid
TIFXGK

SEQ ID NO: 239 - protein, 6 aa, Artificial Sequence
  Synthetic peptide
  MISC_FEATURE (2)..(2): Xaa can be A or V
  misc_feature (3)..(3): Xaa can be any naturally occurring amino acid
  MISC_FEATURE (5)..(5): Xaa can be T or Q
RXXSXH

SEQ ID NO: 240 - protein, 6 aa, Artificial Sequence
  Synthetic peptide
  misc_feature (5)..(5): Xaa can be any naturally occurring amino acid
KWHGXY

SEQ ID NO: 241 - protein, 5 aa, Artificial Sequence
  Synthetic peptide
MPEDK

SEQ ID NO: 242 - protein, 9 aa, Artificial Sequence
  Synthetic peptide
  misc_feature (2)..(4): Xaa can be any naturally occurring amino acid
  MISC_FEATURE (5)..(5): Xaa can be F or Y
  misc_feature (6)..(6): Xaa can be any naturally occurring amino acid
  MISC_FEATURE (7)..(7): Xaa can be A or S
  MISC_FEATURE (9)..(9): Xaa can be N or T
EXXXXXXDX

SEQ ID NO: 243 - protein, 8 aa, Artificial Sequence
  Synthetic peptide
  misc_feature (4)..(5): Xaa can be any naturally occurring amino acid
  misc_feature (7)..(7): Xaa can be any naturally occurring amino acid
  MISC_FEATURE (8)..(8): Xaa can be V or I
NQSXXKXX

SEQ ID NO: 244 - protein, 6 aa, Artificial Sequence
  Synthetic peptide
  misc_feature (2)..(2): Xaa can be any naturally occurring amino acid
  MISC_FEATURE (4)..(4): Xaa can be N, A or S
KXYXPY

SEQ ID NO: 245 - protein, 6 aa, Artificial Sequence
  Synthetic peptide
  MISC_FEATURE (1)..(1): Xaa can be P or Q
  MISC_FEATURE (2)..(2): Xaa can be V or L
XXHPRI

SEQ ID NO: 246 - protein, 7 aa, Artificial Sequence
  Synthetic peptide
  misc_feature (5)..(6): Xaa can be any naturally occurring amino acid
EDGMXXW

SEQ ID NO: 247 - protein, 6 aa, Artificial Sequence
  Synthetic peptide
  misc_feature (4)..(4): Xaa can be any naturally occurring amino acid
YASXQE

SEQ ID NO: 248 - protein, 6 aa, Artificial Sequence
  Synthetic peptide
  misc_feature (3)..(3): Xaa can be any naturally occurring amino acid
  MISC_FEATURE (5)..(5): Xaa can be Q or K
KQXQXE

SEQ ID NO: 249 - protein, 6 aa, Artificial Sequence
  Synthetic peptide
  MISC_FEATURE (2)..(2): Xaa can be A or S
  MISC_FEATURE (6)..(6): Xaa can be I, V or M
KXVFDX

SEQ ID NO: 250 - protein, 6 aa, Artificial Sequence
  Synthetic peptide
  MISC_FEATURE (3)..(3): Xaa can be Q or E
  misc_feature (4)..(4): Xaa can be any naturally occurring amino acid
  MISC_FEATURE (5)..(5): Xaa can be D or N
PNXXXP

SEQ ID NO: 251 - protein, 6 aa, Artificial Sequence
  Synthetic peptide
  MISC_FEATURE (2)..(2): Xaa can be Q or A
  misc_feature (3)..(3): Xaa can be any naturally occurring amino acid
  MISC_FEATURE (5)..(5): Xaa can be D or N
PXXMXI

SEQ ID NO: 252 - protein, 7 aa, Artificial Sequence
  Synthetic peptide
  MISC_FEATURE (1)..(1): Xaa can be W or R
  misc_feature (2)..(2): Xaa can be any naturally occurring amino acid
  MISC_FEATURE (3)..(3): Xaa can be R, K or H
  MISC_FEATURE (4)..(4): Xaa can be S or T
  misc_feature (5)..(5): Xaa can be any naturally occurring amino acid
XXXXXFD

SEQ ID NO: 253 - protein, 7 aa, Artificial Sequence
  Synthetic peptide
  misc_feature (2)..(2): Xaa can be any naturally occurring amino acid
  misc_feature (6)..(6): Xaa can be any naturally occurring amino acid
KXEPGXK

SEQ ID NO: 254 - protein, 5 aa, Artificial Sequence
  Synthetic peptide
DDCLP

SEQ ID NO: 255 - protein, 10 aa, Artificial Sequence
  Synthetic peptide
  misc_feature (2)..(5): Xaa can be any naturally occurring amino acid
  misc_feature (7)..(7): Xaa can be any naturally occurring amino acid
NXXXXGXHLE

SEQ ID NO: 256 - protein, 7 aa, Artificial Sequence
  Synthetic peptide
  misc_feature (2)..(3): Xaa can be any naturally occurring amino acid
DXXHLEG

SEQ ID NO: 257 - protein, 7 aa, Artificial Sequence
  Synthetic peptide
  misc_feature (3)..(4): Xaa can be any naturally occurring amino acid
  MISC_FEATURE (5)..(5): Xaa can be T or S
RPXXXHN

SEQ ID NO: 258 - protein, 6 aa, Artificial Sequence
  Synthetic peptide
  misc_feature (2)..(2): Xaa can be any naturally occurring amino acid
  MISC_FEATURE (5)..(5): Xaa can be I or V
KXHSXY

SEQ ID NO: 259 - protein, 7 aa, Artificial Sequence
  Synthetic peptide
  misc_feature (2)..(2): Xaa can be any naturally occurring amino acid
  misc_feature (5)..(5): Xaa can be any naturally occurring amino acid
  MISC_FEATURE (6)..(6): Xaa can be I or V
KXHSXXS

SEQ ID NO: 260 - protein, 5 aa, Artificial Sequence
  Synthetic peptide
MSGYE

SEQ ID NO: 261 - protein, 6 aa, Artificial Sequence
  Synthetic peptide
  misc_feature (2)..(2): Xaa can be any naturally occurring amino acid
YXIWGP

SEQ ID NO: 262 - protein, 8 aa, Artificial Sequence
  Synthetic peptide
  misc_feature (2)..(3): Xaa can be any naturally occurring amino acid
  misc_feature (5)..(5): Xaa can be any naturally occurring amino acid
  MISC_FEATURE (8)..(8): Xaa can be R or K
RXXWXMNX

SEQ ID NO: 263 - protein, 7 aa, Artificial Sequence
  Synthetic peptide
  misc_feature (3)..(4): Xaa can be any naturally occurring amino acid
  MISC_FEATURE (6)..(6): Xaa can be F or Y
QPXXTXE

SEQ ID NO: 264 - protein, 5 aa, Artificial Sequence
  Synthetic peptide
YGYNQ

SEQ ID NO: 265 - protein, 5 aa, Artificial Sequence
  Synthetic peptide
ARSPN

SEQ ID NO: 266 - protein, 6 aa, Artificial Sequence
  Synthetic peptide
AGSPNR

SEQ ID NO: 267 - protein, 7 aa, Artificial Sequence
  Synthetic peptide
PDGGVMP

SEQ ID NO: 268 - protein, 7 aa, Artificial Sequence
  Synthetic peptide
NPKLGLT

SEQ ID NO: 269 - protein, 6 aa, Artificial Sequence
  Synthetic peptide
GRRPFF

SEQ ID NO: 270 - protein, 9 aa, Artificial Sequence
  Synthetic peptide
  misc_feature (4)..(4): Xaa can be any naturally occurring amino acid
GGGXGAGGG

SEQ ID NO: 271 - protein, 7 aa, Artificial Sequence
  Synthetic peptide
  MISC_FEATURE (3)..(3): Xaa can be P or A
  MISC_FEATURE (6)..(6): Xaa can be G or A
EGXSTXR

SEQ ID NO: 272 - protein, 9 aa, Artificial Sequence
  Synthetic peptide
  misc_feature (2)..(3): Xaa can be any naturally occurring amino acid
  MISC_FEATURE (6)..(6): Xaa can be I, V or L
  MISC_FEATURE (9)..(9): Xaa can be R or K
KXXSCXGCX

SEQ ID NO: 273 - protein, 6 aa, Artificial Sequence
  Synthetic peptide
SCIGCK

SEQ ID NO: 274 - protein, 4 aa, Artificial Sequence
  Synthetic peptide
CIGC

SEQ ID NO: 275 - protein, 6 aa, Artificial Sequence
  Synthetic peptide
  misc_feature (2)..(2): Xaa can be any naturally occurring amino acid
VXLPHW

SEQ ID NO: 276 - protein, 4 aa, Artificial Sequence
  Synthetic peptide
LPHW

SEQ ID NO: 277 - protein, 7 aa, Artificial Sequence
  Synthetic peptide
  MISC_FEATURE (5)..(5): Xaa can be G or A
  MISC_FEATURE (5)..(5): Xaa can be G or A
PQDTXPR

SEQ ID NO: 278 - protein, 6 aa, Artificial Sequence
  Synthetic peptide
GPPWWP

SEQ ID NO: 279 - protein, 8 aa, Artificial Sequence
  Synthetic peptide
  misc_feature (6)..(6): Xaa can be any naturally occurring amino acid
QQPTTXGW

SEQ ID NO: 280 - protein, 8 aa, Artificial Sequence
  Synthetic peptide
  MISC_FEATURE (1)..(1): Xaa can be L, M, I or V
  misc_feature (4)..(4): Xaa can be any naturally occurring amino acid
XFDXDWYP

SEQ ID NO: 281 - protein, 6 aa, Artificial Sequence
  Synthetic peptide
GRRPFF

SEQ ID NO: 282 - protein, 9 aa, Artificial Sequence
  Synthetic peptide
GGGAGAGGG

SEQ ID NO: 283 - protein, 8 aa, Artificial Sequence
  Synthetic peptide
EGPSTGPR

SEQ ID NO: 284 - protein, 9 aa, Artificial Sequence
  Synthetic peptide
KRPSCIGCK

SEQ ID NO: 285 - protein, 11 aa, Artificial Sequence
  Synthetic peptide
KEVKLPHWTPT

SEQ ID NO: 286 - protein, 7 aa, Artificial Sequence
  Synthetic peptide
PQDTAPR

SEQ ID NO: 287 - protein, 6 aa, Artificial Sequence
  Synthetic peptide
GPPWWP

SEQ ID NO: 288 - protein, 8 aa, Artificial Sequence
  Synthetic peptide
QQPTTEGH

SEQ ID NO: 289 - protein, 8 aa, Artificial Sequence
  Synthetic peptide
LFPDDWYP

SEQ ID NO: 290 - protein, 7 aa, Artificial Sequence
  Synthetic peptide
  misc_feature (2)..(2): Xaa can be any naturally occurring amino acid
  misc_feature (4)..(4): Xaa can be any naturally occurring amino acid
CXGXLIC

SEQ ID NO: 291 - protein, 8 aa, Artificial Sequence
  Synthetic peptide
  misc_feature (2)..(3): Xaa can be any naturally occurring amino acid
  misc_feature (5)..(5): Xaa can be any naturally occurring amino acid
  MISC_FEATURE (6)..(6): Xaa can be I or V
  MISC_FEATURE (8)..(8): Xaa can be I or V
CXXKXXCX

SEQ ID NO: 292 - protein, 9 aa, Artificial Sequence
  Synthetic peptide
  MISC_FEATURE (2)..(2): Xaa can be G, A or S
  misc_feature (4)..(4): Xaa can be any naturally occurring amino acid
  misc_feature (6)..(8): Xaa can be any naturally occurring amino acid
WXCXGXXXC

SEQ ID NO: 293 - protein, 5 aa, Artificial Sequence
  Synthetic peptide
  MISC_FEATURE (1)..(1): Xaa can be R or K
  MISC_FEATURE (4)..(4): Xaa can be I or V
XKLXE

SEQ ID NO: 294 - protein, 5 aa, Artificial Sequence
  Synthetic peptide
KLIMT

SEQ ID NO: 295 - protein, 7 aa, Artificial Sequence
  Synthetic peptide
  MISC_FEATURE (1)..(1): Xaa can be Q or E
  misc_feature (2)..(3): Xaa can be any naturally occurring amino acid
XXXPFRY

SEQ ID NO: 296 - protein, 8 aa, Artificial Sequence
  Synthetic peptide
  misc_feature (2)..(3): Xaa can be any naturally occurring amino acid
  misc_feature (5)..(5): Xaa can be any naturally occurring amino acid
  MISC_FEATURE (6)..(6): Xaa can be I or V
  MISC_FEATURE (8)..(8): Xaa can be I or V
CXXKXXCX

SEQ ID NO: 297 - protein, 7 aa, Artificial Sequence
  Synthetic peptide
  MISC_FEATURE (1)..(1): Xaa can be L or F
  misc_feature (2)..(3): Xaa can be any naturally occurring amino acid
  MISC_FEATURE (4)..(4): Xaa can be L, I or V
  MISC_FEATURE (5)..(5): Xaa can be N or D
XXXXXKW

SEQ ID NO: 298 - protein, 5 aa, Artificial Sequence
  Synthetic peptide
  MISC_FEATURE (1)..(1): Xaa can be A or P
  MISC_FEATURE (2)..(2): Xaa can be G or C
XXGFG

SEQ ID NO: 299 - protein, 6 aa, Artificial Sequence
  Synthetic peptide
  misc_feature (3)..(3): Xaa can be any naturally occurring amino acid
  MISC_FEATURE (4)..(4): Xaa can be T or S
LIXXTY

SEQ ID NO: 300 - protein, 7 aa, Artificial Sequence
  Synthetic peptide
  MISC_FEATURE (1)..(1): Xaa can be R or K
  misc_feature (4)..(5): Xaa can be any naturally occurring amino acid
  MISC_FEATURE (6)..(6): Xaa can be M or V
XKLXXXY

SEQ ID NO: 301 - protein, 5 aa, Artificial Sequence
  Synthetic peptide
  MISC_FEATURE (3)..(3): Xaa can be G or A
  MISC_FEATURE (4)..(4): Xaa can be A or Q
  MISC_FEATURE (5)..(5): Xaa can be A, Y or V
GFXXX

SEQ ID NO: 302 - protein, 6 aa, Artificial Sequence
  Synthetic peptide
  MISC_FEATURE (4)..(4): Xaa can be R or Q
  misc_feature (5)..(5): Xaa can be any naturally occurring amino acid
  MISC_FEATURE (6)..(6): Xaa can be F, N or Y
GFGXXX

SEQ ID NO: 303 - protein, 6 aa, Artificial Sequence
  Synthetic peptide
  MISC_FEATURE (1)..(1): Xaa can be K or R
  misc_feature (3)..(3): Xaa can be any naturally occurring amino acid
  MISC_FEATURE (6)..(6): Xaa can be V, I or M
XKXIHX

SEQ ID NO: 304 - protein, 5 aa, Artificial Sequence
  Synthetic peptide
  MISC_FEATURE (2)..(2): Xaa can be I or V
RXPFG

SEQ ID NO: 305 - protein, 7 aa, Artificial Sequence
  Synthetic peptide
  misc_feature (4)..(5): Xaa can be any naturally occurring amino acid
  MISC_FEATURE (6)..(6): Xaa can be T or Y
KLIXXXT

SEQ ID NO: 306 - protein, 7 aa, Artificial Sequence
  Synthetic peptide
CSGKLIC

SEQ ID NO: 307 - protein, 8 aa, Artificial Sequence
  Synthetic peptide
CSGKLICT

SEQ ID NO: 308 - protein, 9 aa, Artificial Sequence
  Synthetic peptide
WGCSGKLIC

SEQ ID NO: 309 - protein, 8 aa, Artificial Sequence
  Synthetic peptide
CSGKLICT

SEQ ID NO: 310 - protein, 7 aa, Artificial Sequence
  Synthetic peptide
LLALDKW

SEQ ID NO: 311 - protein, 5 aa, Artificial Sequence
  Synthetic peptide
AVGMG

SEQ ID NO: 312 - protein, 5 aa, Artificial Sequence
  Synthetic peptide
LICTT

SEQ ID NO: 313 - protein, 5 aa, Artificial Sequence
  Synthetic peptide
GFGAV

SEQ ID NO: 314 - protein, 6 aa, Artificial Sequence
  Synthetic peptide
RKGIRI

SEQ ID NO: 315 - protein, 6 aa, Artificial Sequence
  Synthetic peptide
KKGIAI

SEQ ID NO: 316 - protein, 6 aa, Artificial Sequence
  Synthetic peptide
RKGIHM

SEQ ID NO: 317 - protein, 6 aa, Artificial Sequence
  Synthetic peptide
RKSIHM

SEQ ID NO: 318 - protein, 6 aa, Artificial Sequence
  Synthetic peptide
KLICTT

SEQ ID NO: 319 - protein, 8 aa, Artificial Sequence
  Synthetic peptide
  misc_feature (3)..(4): Xaa can be any naturally occurring amino acid
  misc_feature (6)..(6): Xaa can be any naturally occurring amino acid
VRXXYXQH

SEQ ID NO: 320 - protein, 9 aa, Artificial Sequence
  Synthetic peptide
  misc_feature (4)..(6): Xaa can be any naturally occurring amino acid
  misc_feature (8)..(8): Xaa can be any naturally occurring amino acid
CEDXXXHXC

SEQ ID NO: 321 - protein, 7 aa, Artificial Sequence
  Synthetic peptide
  misc_feature (5)..(6): Xaa can be any naturally occurring amino acid
DAEQXXR

SEQ ID NO: 322 - protein, 5 aa, Artificial Sequence
  Synthetic peptide
WPGIF

SEQ ID NO: 323 - protein, 6 aa, Artificial Sequence
  Synthetic peptide
  misc_feature (5)..(5): Xaa can be any naturally occurring amino acid
CCYDXE

SEQ ID NO: 324 - protein, 7 aa, Artificial Sequence
  Synthetic peptide
  misc_feature (2)..(2): Xaa can be any naturally occurring amino acid
  misc_feature (6)..(6): Xaa can be any naturally occurring amino acid
LXPDNXT

SEQ ID NO: 325 - protein, 7 aa, Artificial Sequence
  Synthetic peptide
  misc_feature (2)..(2): Xaa can be any naturally occurring amino acid
  misc_feature (6)..(6): Xaa can be any naturally occurring amino acid
FXWGQXY

SEQ ID NO: 326 - protein, 10 aa, Artificial Sequence
  Synthetic peptide
  misc_feature (2)..(2): Xaa can be any naturally occurring amino acid
  misc_feature (6)..(9): Xaa can be any naturally occurring amino acid
KXEGHXXXXA

SEQ ID NO: 327 - protein, 9 aa, Artificial Sequence
  Synthetic peptide
  misc_feature (2)..(3): Xaa can be any naturally occurring amino acid
  misc_feature (5)..(5): Xaa can be any naturally occurring amino acid
  misc_feature (8)..(8): Xaa can be any naturally occurring amino acid
CXXGXCQXK

SEQ ID NO: 328 - protein, 8 aa, Artificial Sequence
  Synthetic peptide
  misc_feature (3)..(3): Xaa can be any naturally occurring amino acid
  misc_feature (5)..(6): Xaa can be any naturally occurring amino acid
  MISC_FEATURE (7)..(7): Xaa can be D or E
  MISC_FEATURE (8)..(8): Xaa can be E or D
CCXDXXXX

SEQ ID NO: 329 - protein, 6 aa, Artificial Sequence
  Synthetic peptide
  misc_feature (4)..(4): Xaa can be any naturally occurring amino acid
RNGXED

SEQ ID NO: 330 - protein, 8 aa, Artificial Sequence
  Synthetic peptide
  MISC_FEATURE (1)..(1): Xaa can be D or E
  misc_feature (2)..(2): Xaa can be any naturally occurring amino acid
  misc_feature (4)..(4): Xaa can be any naturally occurring amino acid
  misc_feature (7)..(7): Xaa can be any naturally occurring amino acid
XXRXIYXQ

SEQ ID NO: 331 - protein, 6 aa, Artificial Sequence
  Synthetic peptide
  misc_feature (2)..(2): Xaa can be any naturally occurring amino acid
WXRCGL

SEQ ID NO: 332 - protein, 10 aa, Artificial Sequence
  Synthetic peptide
  MISC_FEATURE (2)..(2): Xaa can be E or D
  misc_feature (3)..(3): Xaa can be any naturally occurring amino acid
  misc_feature (5)..(6): Xaa can be any naturally occurring amino acid
  misc_feature (8)..(9): Xaa can be any naturally occurring amino acid
DXXRXXYXXH

SEQ ID NO: 333 - protein, 7 aa, Artificial Sequence
  Synthetic peptide
  misc_feature (3)..(3): Xaa can be any naturally occurring amino acid
  misc_feature (5)..(5): Xaa can be any naturally occurring amino acid
  MISC_FEATURE (6)..(6): Xaa can be A or V
WCXLXXN

SEQ ID NO: 334 - protein, 6 aa, Artificial Sequence
  Synthetic peptide
  misc_feature (2)..(2): Xaa can be any naturally occurring amino acid
LXTPWI

SEQ ID NO: 335 - protein, 8 aa, Artificial Sequence
  Synthetic peptide
  misc_feature (3)..(5): Xaa can be any naturally occurring amino acid
  MISC_FEATURE (8)..(8): Xaa can be C or A
CWXXXGLX

SEQ ID NO: 336 - protein, 5 aa, Artificial Sequence
  Synthetic peptide
  MISC_FEATURE (3)..(3): Xaa can be A or V
IDXEP

SEQ ID NO: 337 - protein, 6 aa, Artificial Sequence
  Synthetic peptide
  MISC_FEATURE (3)..(3): Xaa can be N or K
  MISC_FEATURE (4)..(4): Xaa can be V or T
  misc_feature (5)..(5): Xaa can be any naturally occurring amino acid
HFXXXK

SEQ ID NO: 338 - protein, 7 aa, Artificial Sequence
  Synthetic peptide
  misc_feature (2)..(2): Xaa can be any naturally occurring amino acid
  misc_feature (6)..(6): Xaa can be any naturally occurring amino acid
QXNHQXK

SEQ ID NO: 339 - protein, 6 aa, Artificial Sequence
  Synthetic peptide
  misc_feature (3)..(3): Xaa can be any naturally occurring amino acid
FEXKEP

SEQ ID NO: 340 - protein, 4 aa, Artificial Sequence
  Synthetic peptide
  MISC_FEATURE (1)..(1): Xaa can be F, Y or W
  MISC_FEATURE (4)..(4): Xaa can be V or I
XDAX

SEQ ID NO: 341 - protein, 5 aa, Artificial Sequence
  Synthetic peptide
DFDKR

SEQ ID NO: 342 - protein, 4 aa, Artificial Sequence
  Synthetic peptide
WETC

SEQ ID NO: 343 - protein, 5 aa, Artificial Sequence
  Synthetic peptide
KLDGP

SEQ ID NO: 344 - protein, 6 aa, Artificial Sequence
  Synthetic peptide
  misc_feature (5)..(5): Xaa can be any naturally occurring amino acid
WIYPXK

SEQ ID NO: 345 - protein, 5 aa, Artificial Sequence
  Synthetic peptide
  MISC_FEATURE (2)..(2): Xaa can be H or S
VXDSK

SEQ ID NO: 346 - protein, 5 aa, Artificial Sequence
  Synthetic peptide
EQCGT

SEQ ID NO: 347 - protein, 5 aa, Artificial Sequence
  Synthetic peptide
  MISC_FEATURE (1)..(1): Xaa can be K or E
  MISC_FEATURE (2)..(2): Xaa can be M, V, I or T
XXPYA

SEQ ID NO: 348 - protein, 7 aa, Artificial Sequence
  Synthetic peptide
  MISC_FEATURE (1)..(1): Xaa can be D or E
  misc_feature (2)..(3): Xaa can be any naturally occurring amino acid
  MISC_FEATURE (6)..(6): Xaa can be R or P
XXXMLXW

SEQ ID NO: 349 - protein, 7 aa, Artificial Sequence
  Synthetic peptide
  misc_feature (3)..(3): Xaa can be any naturally occurring amino acid
  misc_feature (6)..(6): Xaa can be any naturally occurring amino acid
  MISC_FEATURE (7)..(7): Xaa can be F or Y
YEXLHXX

SEQ ID NO: 350 - protein, 6 aa, Artificial Sequence
  Synthetic peptide
  MISC_FEATURE (3)..(3): Xaa can be T, S or N
  misc_feature (4)..(4): Xaa can be any naturally occurring amino acid
WYXXEK

SEQ ID NO: 351 - protein, 5 aa, Artificial Sequence
  Synthetic peptide
  MISC_FEATURE: Xaa can be Y or F
  misc_feature (1)..(1): Xaa can be any naturally occurring amino acid
  MISC_FEATURE (3)..(3): Xaa can be D, N or S
XHXAV

SEQ ID NO: 352 - protein, 6 aa, Artificial Sequence
  Synthetic peptide
  misc_feature (2)..(2): Xaa can be any naturally occurring amino acid
  MISC_FEATURE (5)..(5): Xaa can be V or I
DXTGXP

SEQ ID NO: 353 - protein, 7 aa, Artificial Sequence
  Synthetic peptide
  misc_feature (3)..(4): Xaa can be any naturally occurring amino acid
  MISC_FEATURE (6)..(6): Xaa can be A or V
FDXXGEH

SEQ ID NO: 354 - protein, 7 aa, Artificial Sequence
  Synthetic peptide
  MISC_FEATURE (3)..(3): Xaa can be A or K
  misc_feature (4)..(5): Xaa can be any naturally occurring amino acid
  MISC_FEATURE (6)..(6): Xaa can be H or E
QCXXXXC

SEQ ID NO: 355 - protein, 7 aa, Artificial Sequence
  Synthetic peptide
  MISC_FEATURE (3)..(3): Xaa can be F or Y
  misc_feature (4)..(4): Xaa can be any naturally occurring amino acid
  misc_feature (6)..(6): Xaa can be any naturally occurring amino acid
LWXXPXE

SEQ ID NO: 356 - protein, 7 aa, Artificial Sequence
  Synthetic peptide
  MISC_FEATURE (2)..(2): Xaa can be M or I
  MISC_FEATURE (3)..(3): Xaa can be P or A
  misc_feature (5)..(6): Xaa can be any naturally occurring amino acid
CXXGXXC

SEQ ID NO: 357 - protein, 9 aa, Artificial Sequence
  Synthetic peptide
  misc_feature (2)..(5): Xaa can be any naturally occurring amino acid
  MISC_FEATURE (6)..(6): Xaa can be A, V or S
CXXXXXADC

SEQ ID NO: 358 - protein, 10 aa, Artificial Sequence
  Synthetic peptide
  misc_feature (5)..(9): Xaa can be any naturally occurring amino acid
VQQEXXXXXP

SEQ ID NO: 359 - protein, 9 aa, Artificial Sequence
  Synthetic peptide
  misc_feature (5)..(8): Xaa can be any naturally occurring amino acid
  MISC_FEATURE (9)..(9): Xaa can be Y or C
QQEGXXXXX

SEQ ID NO: 360 - protein, 5 aa, Artificial Sequence
  Synthetic peptide
  MISC_FEATURE (4)..(4): Xaa can be I or V
QEGXQ

SEQ ID NO: 361 - protein, 6 aa, Artificial Sequence
  Synthetic peptide
  MISC_FEATURE (2)..(2): Xaa can be I or V
  misc_feature (4)..(4): Xaa can be any naturally occurring amino acid
GXQXEG

SEQ ID NO: 362 - protein, 9 aa, Artificial Sequence
  Synthetic peptide
  MISC_FEATURE (1)..(1): Xaa can be L or I
  misc_feature (2)..(3): Xaa can be any naturally occurring amino acid
  MISC_FEATURE (5)..(5): Xaa can be I, L or V
  misc_feature (6)..(7): Xaa can be any naturally occurring amino acid
XXXAXXXRG

SEQ ID NO: 363 - protein, 10 aa, Artificial Sequence
  Synthetic peptide
  MISC_FEATURE (1)..(1): Xaa can be A, T, N, S or  D
  misc_feature (2)..(5): Xaa can be any naturally occurring amino acid
  MISC_FEATURE (8)..(8): Xaa can be L, A or M
  misc_feature (9)..(9): Xaa can be any naturally occurring amino acid
XXXXXAIXXR

SEQ ID NO: 364 - protein, 8 aa, Artificial Sequence
  Synthetic peptide
  misc_feature (2)..(2): Xaa can be any naturally occurring amino acid
  MISC_FEATURE (3)..(3): Xaa can be L or M
  misc_feature (4)..(4): Xaa can be any naturally occurring amino acid
  misc_feature (7)..(7): Xaa can be any naturally occurring amino acid
IXXXGFXK

SEQ ID NO: 365 - protein, 6 aa, Artificial Sequence
  Synthetic peptide
  misc_feature (2)..(2): Xaa can be any naturally occurring amino acid
  MISC_FEATURE (5)..(5): Xaa can be R or Q
LXGMXK

SEQ ID NO: 366 - protein, 8 aa, Artificial Sequence
  Synthetic peptide
  MISC_FEATURE (1)..(1): Xaa can be H or R
  misc_feature (2)..(2): Xaa can be any naturally occurring amino acid
  misc_feature (4)..(4): Xaa can be any naturally occurring amino acid
  misc_feature (7)..(7): Xaa can be any naturally occurring amino acid
XXDXTNXF

SEQ ID NO: 367 - protein, 5 aa, Artificial Sequence
  Synthetic peptide
  MISC_FEATURE (1)..(1): Xaa can be D or A
XDPTN

SEQ ID NO: 368 - protein, 8 aa, Artificial Sequence
  Synthetic peptide
  MISC_FEATURE (1)..(1): Xaa can be K or R
  misc_feature (2)..(2): Xaa can be any naturally occurring amino acid
  MISC_FEATURE (3)..(3): Xaa can be D or E
  misc_feature (4)..(4): Xaa can be any naturally occurring amino acid
  misc_feature (7)..(7): Xaa can be any naturally occurring amino acid
XXXXTNXF

SEQ ID NO: 369 - protein, 5 aa, Artificial Sequence
  Synthetic peptide
  MISC_FEATURE (1)..(1): Xaa can be E or T
  MISC_FEATURE (2)..(2): Xaa can be M or L
XXHKF

SEQ ID NO: 370 - protein, 7 aa, Artificial Sequence
  Synthetic peptide
  MISC_FEATURE (1)..(1): Xaa can be M or L
  misc_feature (2)..(3): Xaa can be any naturally occurring amino acid
XXXEFHK

SEQ ID NO: 371 - protein, 10 aa, Artificial Sequence
  Synthetic peptide
  MISC_FEATURE (2)..(2): Xaa can be T or I
  misc_feature (5)..(9): Xaa can be any naturally occurring amino acid
QXEQXXXXXK

SEQ ID NO: 372 - protein, 6 aa, Artificial Sequence
  Synthetic peptide
  misc_feature (2)..(2): Xaa can be any naturally occurring amino acid
  MISC_FEATURE (5)..(5): Xaa can be I or L
DXSPXE

SEQ ID NO: 373 - protein, 7 aa, Artificial Sequence
  Synthetic peptide
  misc_feature (3)..(3): Xaa can be any naturally occurring amino acid
  MISC_FEATURE (4)..(4): Xaa can be A or P
  misc_feature (6)..(6): Xaa can be any naturally occurring amino acid
PFXXYXK

SEQ ID NO: 374 - protein, 10 aa, Artificial Sequence
  Synthetic peptide
  misc_feature (2)..(3): Xaa can be any naturally occurring amino acid
  misc_feature (6)..(7): Xaa can be any naturally occurring amino acid
  MISC_FEATURE (8)..(8): Xaa can be L or V
  misc_feature (9)..(9): Xaa can be any naturally occurring amino acid
VXXYFXXXXK

SEQ ID NO: 375 - protein, 7 aa, Artificial Sequence
  Synthetic peptide
  misc_feature (2)..(2): Xaa can be any naturally occurring amino acid
  misc_feature (5)..(5): Xaa can be any naturally occurring amino acid
KXVDXDR

SEQ ID NO: 376 - protein, 5 aa, Artificial Sequence
  Synthetic peptide
  MISC_FEATURE (1)..(1): Xaa can be D or N
  MISC_FEATURE (2)..(2): Xaa can be A or S
  MISC_FEATURE (4)..(4): Xaa can be A or G
XXAXF

SEQ ID NO: 377 - protein, 7 aa, Artificial Sequence
  Synthetic peptide
  misc_feature (2)..(2): Xaa can be any naturally occurring amino acid
  MISC_FEATURE (3)..(3): Xaa can be N or A
  misc_feature (4)..(4): Xaa can be any naturally occurring amino acid
CXXXKFC

SEQ ID NO: 378 - protein, 6 aa, Artificial Sequence
  Synthetic peptide
  misc_feature (2)..(2): Xaa can be any naturally occurring amino acid
  MISC_FEATURE (3)..(3): Xaa can be G, R, S or T
  MISC_FEATURE (6)..(6): Xaa can be Y or F
KXXAEX

SEQ ID NO: 379 - protein, 8 aa, Artificial Sequence
  Synthetic peptide
  MISC_FEATURE (4)..(4): Xaa can be P or A
  misc_feature (5)..(7): Xaa can be any naturally occurring amino acid
  MISC_FEATURE (8)..(8): Xaa can be D, H or E
HQVXXXXX

SEQ ID NO: 380 - protein, 9 aa, Artificial Sequence
  Synthetic peptide
  misc_feature (3)..(4): Xaa can be any naturally occurring amino acid
  MISC_FEATURE (6)..(6): Xaa can be I or F
  MISC_FEATURE (6)..(6)
  misc_feature (7)..(8): Xaa can be any naturally occurring amino acid
IPXXVXXXR

SEQ ID NO: 381 - protein, 8 aa, Artificial Sequence
  Synthetic peptide
  misc_feature (2)..(2): Xaa can be any naturally occurring amino acid
  MISC_FEATURE (3)..(3): Xaa can be A, L or T
  misc_feature (4)..(4): Xaa can be any naturally occurring amino acid
  misc_feature (7)..(7): Xaa can be any naturally occurring amino acid
  MISC_FEATURE (8)..(8): Xaa can be C or A
CXXXWEXX

SEQ ID NO: 382 - protein, 10 aa, Artificial Sequence
  Synthetic peptide
  misc_feature (2)..(4): Xaa can be any naturally occurring amino acid
  MISC_FEATURE (7)..(7): Xaa can be I or L
  misc_feature (8)..(9): Xaa can be any naturally occurring amino acid
CXXXCAXXXR

SEQ ID NO: 383 - protein, 8 aa, Artificial Sequence
  Synthetic peptide
  MISC_FEATURE (2)..(2): Xaa can be I or V
  misc_feature (4)..(5): Xaa can be any naturally occurring amino acid
  MISC_FEATURE (6)..(6): Xaa can be M or T
  misc_feature (7)..(7): Xaa can be any naturally occurring amino acid
IXIXXXXK

SEQ ID NO: 384 - protein, 6 aa, Artificial Sequence
  Synthetic peptide
  MISC_FEATURE (3)..(3): Xaa can be I, T or L
  misc_feature (4)..(4): Xaa can be any naturally occurring amino acid
  MISC_FEATURE (5)..(5): Xaa can be K or N
  MISC_FEATURE (6)..(6): Xaa can be F or Y
QGXXXX

SEQ ID NO: 385 - protein, 8 aa, Artificial Sequence
  Synthetic peptide
  misc_feature (2)..(3): Xaa can be any naturally occurring amino acid
  misc_feature (6)..(6): Xaa can be any naturally occurring amino acid
KXXPPXIN

SEQ ID NO: 386 - protein, 7 aa, Artificial Sequence
  Synthetic peptide
  MISC_FEATURE (2)..(2): Xaa can be Y or F
  MISC_FEATURE (3)..(3): Xaa can be F or Y
  misc_feature (5)..(6): Xaa can be any naturally occurring amino acid
GXXFXXK

SEQ ID NO: 387 - protein, 6 aa, Artificial Sequence
  Synthetic peptide
  misc_feature (5)..(5): Xaa can be any naturally occurring amino acid
  MISC_FEATURE (6)..(6): Xaa  can be I or V
DKNVXX

SEQ ID NO: 388 - protein, 6 aa, Artificial Sequence
  Synthetic peptide
  MISC_FEATURE (1)..(1): Xaa can be Q or E
  MISC_FEATURE (2)..(2): Xaa can be K or R
  MISC_FEATURE (3)..(3): Xaa can be N or D
  misc_feature (4)..(4): Xaa can be any naturally occurring amino acid
XXXXSG

SEQ ID NO: 389 - protein, 5 aa, Artificial Sequence
  Synthetic peptide
  MISC_FEATURE (2)..(2): Xaa can be R or K
KXPGD

SEQ ID NO: 390 - protein, 6 aa, Artificial Sequence
  Synthetic peptide
  misc_feature (4)..(4): Xaa can be any naturally occurring amino acid
EGAXQP

SEQ ID NO: 391 - protein, 5 aa, Artificial Sequence
  Synthetic peptide
GSPEY

SEQ ID NO: 392 - protein, 10 aa, Artificial Sequence
  Synthetic peptide
VQQEGAQQQP

SEQ ID NO: 393 - protein, 5 aa, Artificial Sequence
  Synthetic peptide
QEGVQ

SEQ ID NO: 394 - protein, 6 aa, Artificial Sequence
  Synthetic peptide
GVQQEG

SEQ ID NO: 395 - protein, 9 aa, Artificial Sequence
  Synthetic peptide
ILKAVVERG

SEQ ID NO: 396 - protein, 9 aa, Artificial Sequence
  Synthetic peptide
IAAAIVLRG

SEQ ID NO: 397 - protein, 10 aa, Artificial Sequence
  Synthetic peptide
DQIAAAIALR

SEQ ID NO: 398 - protein, 10 aa, Artificial Sequence
  Synthetic peptide
AKKMRAILVR

SEQ ID NO: 399 - protein, 10 aa, Artificial Sequence
  Synthetic peptide
AENHKAILFR

SEQ ID NO: 400 - protein, 8 aa, Artificial Sequence
  Synthetic peptide
IKLPGFKK

SEQ ID NO: 401 - protein, 8 aa, Artificial Sequence
  Synthetic peptide
IFLEGFLK

SEQ ID NO: 402 - protein, 6 aa, Artificial Sequence
  Synthetic peptide
LRGMRK

SEQ ID NO: 403 - protein, 5 aa, Artificial Sequence
  Synthetic peptide
DDPTN

SEQ ID NO: 404 - protein, 8 aa, Artificial Sequence
  Synthetic peptide
KTDRTNDF

SEQ ID NO: 405 - protein, 8 aa, Artificial Sequence
  Synthetic peptide
KDDPTNKF

SEQ ID NO: 406 - protein, 8 aa, Artificial Sequence
  Synthetic peptide
KTDKTNDF

SEQ ID NO: 407 - protein, 5 aa, Artificial Sequence
  Synthetic peptide
TLHKF

SEQ ID NO: 408 - protein, 10 aa, Artificial Sequence
  Synthetic peptide
QTEQSSTSTK

SEQ ID NO: 409 - protein, 6 aa, Artificial Sequence
  Synthetic peptide
DLSPIE

SEQ ID NO: 410 - protein, 7 aa, Artificial Sequence
  Synthetic peptide
PFSAYIK

SEQ ID NO: 411 - protein, 10 aa, Artificial Sequence
  Synthetic peptide
VKDYFDSLAK

SEQ ID NO: 412 - protein, 5 aa, Artificial Sequence
  Synthetic peptide
DAAAF

SEQ ID NO: 413 - protein, 6 aa, Artificial Sequence
  Synthetic peptide
KFRAEF

SEQ ID NO: 414 - protein, 6 aa, Artificial Sequence
  Synthetic peptide
KSSAEF

SEQ ID NO: 415 - protein, 6 aa, Artificial Sequence
  Synthetic peptide
KGGAEF

SEQ ID NO: 416 - protein, 8 aa, Artificial Sequence
  Synthetic peptide
IIIIDTSK

SEQ ID NO: 417 - protein, 8 aa, Artificial Sequence
  Synthetic peptide
IIINGMTK

SEQ ID NO: 418 - protein, 8 aa, Artificial Sequence
  Synthetic peptide
IIITNMEK

SEQ ID NO: 419 - protein, 6 aa, Artificial Sequence
  Synthetic peptide
QGIINY

SEQ ID NO: 420 - protein, 6 aa, Artificial Sequence
  Synthetic peptide
QGICNY

SEQ ID NO: 421 - protein, 8 aa, Artificial Sequence
  Synthetic peptide
KETPPALN

SEQ ID NO: 422 - protein, 7 aa, Artificial Sequence
  Synthetic peptide
GFYFIFK

SEQ ID NO: 423 - protein, 6 aa, Artificial Sequence
  Synthetic peptide
DKNVKI

SEQ ID NO: 424 - protein, 6 aa, Artificial Sequence
  Synthetic peptide
EKNSSG

SEQ ID NO: 425 - protein, 5 aa, Artificial Sequence
  Synthetic peptide
KKPGD

SEQ ID NO: 426 - protein, 6 aa, Artificial Sequence
  Synthetic peptide
EGAQQP

SEQ ID NO: 427 - protein, 5 aa, Artificial Sequence
  Synthetic peptide
GSPEY

SEQ ID NO: 428 - protein, 6 aa, Artificial Sequence
  Synthetic peptide
HEHEFQ

SEQ ID NO: 429 - protein, 6 aa, Artificial Sequence
  Synthetic peptide
LDFWRE

SEQ ID NO: 430 - protein, 6 aa, Artificial Sequence
  Synthetic peptide
LDFWQE

SEQ ID NO: 431 - protein, 6 aa, Artificial Sequence
  Synthetic peptide
LDMWEE

SEQ ID NO: 432 - protein, 5 aa, Artificial Sequence
  Synthetic peptide
HCSAC

SEQ ID NO: 433 - protein, 6 aa, Artificial Sequence
  Synthetic peptide
FSGVVN

SEQ ID NO: 434 - protein, 6 aa, Artificial Sequence
  Synthetic peptide
YPGVVN

SEQ ID NO: 435 - protein, 9 aa, Artificial Sequence
  Synthetic peptide
KGSHGRGFI

SEQ ID NO: 436 - protein, 5 aa, Artificial Sequence
  Synthetic peptide
GPHAE

SEQ ID NO: 437 - protein, 5 aa, Artificial Sequence
  Synthetic peptide
PRREP

SEQ ID NO: 438 - protein, 6 aa, Artificial Sequence
  Synthetic peptide
PVPDFS

SEQ ID NO: 439 - protein, 6 aa, Artificial Sequence
  Synthetic peptide
PVPDFT

SEQ ID NO: 440 - protein, 6 aa, Artificial Sequence
  Synthetic peptide
PLPDFT

SEQ ID NO: 441 - protein, 6 aa, Artificial Sequence
  Synthetic peptide
PLPDFS

SEQ ID NO: 442 - protein, 6 aa, Artificial Sequence
  Synthetic peptide
PAPDFS

SEQ ID NO: 443 - protein, 10 aa, Artificial Sequence
  Synthetic peptide
NAGLEVYAED

SEQ ID NO: 444 - protein, 10 aa, Artificial Sequence
  Synthetic peptide
NRRRERYGED

SEQ ID NO: 445 - protein, 7 aa, Artificial Sequence
  Synthetic peptide
PGAVLLD

SEQ ID NO: 446 - protein, 7 aa, Artificial Sequence
  Synthetic peptide
PAASKLD

SEQ ID NO: 447 - protein, 7 aa, Artificial Sequence
  Synthetic peptide
PAAESLD

SEQ ID NO: 448 - protein, 7 aa, Artificial Sequence
  Synthetic peptide
PGAARLD

SEQ ID NO: 449 - protein, 7 aa, Artificial Sequence
  Synthetic peptide
PGALDLD

SEQ ID NO: 450 - protein, 7 aa, Artificial Sequence
  Synthetic peptide
MPSWSNE

SEQ ID NO: 451 - protein, 7 aa, Artificial Sequence
  Synthetic peptide
MPSTSDE

SEQ ID NO: 452 - protein, 7 aa, Artificial Sequence
  Synthetic peptide
MPSESTE

SEQ ID NO: 453 - protein, 7 aa, Artificial Sequence
  Synthetic peptide
MPSASPE

SEQ ID NO: 454 - protein, 7 aa, Artificial Sequence
  Synthetic peptide
RLYVHRS

SEQ ID NO: 455 - protein, 7 aa, Artificial Sequence
  Synthetic peptide
RLYRHRT

SEQ ID NO: 456 - protein, 7 aa, Artificial Sequence
  Synthetic peptide
KGYFHRT

SEQ ID NO: 457 - protein, 8 aa, Artificial Sequence
  Synthetic peptide
KPPFEFGK

SEQ ID NO: 458 - protein, 8 aa, Artificial Sequence
  Synthetic peptide
KPGFVFLK

SEQ ID NO: 459 - protein, 7 aa, Artificial Sequence
  Synthetic peptide
DDSEGAR

SEQ ID NO: 460 - protein, 7 aa, Artificial Sequence
  Synthetic peptide
DDSCGRR

SEQ ID NO: 461 - protein, 7 aa, Artificial Sequence
  Synthetic peptide
DDSKGDR

SEQ ID NO: 462 - protein, 7 aa, Artificial Sequence
  Synthetic peptide
DDSSGYR

SEQ ID NO: 463 - protein, 7 aa, Artificial Sequence
  Synthetic peptide
KEAAGRG

SEQ ID NO: 464 - protein, 7 aa, Artificial Sequence
  Synthetic peptide
KDASLRG

SEQ ID NO: 465 - protein, 7 aa, Artificial Sequence
  Synthetic peptide
KGSSGRG

SEQ ID NO: 466 - protein, 7 aa, Artificial Sequence
  Synthetic peptide
KTSSRRG

SEQ ID NO: 467 - protein, 7 aa, Artificial Sequence
  Synthetic peptide
KTQTVRG

SEQ ID NO: 468 - protein, 7 aa, Artificial Sequence
  Synthetic peptide
KRSTLRG

SEQ ID NO: 469 - protein, 5 aa, Artificial Sequence
  Synthetic peptide
DQPEN

SEQ ID NO: 470 - protein, 5 aa, Artificial Sequence
  Synthetic peptide
GQPEN

SEQ ID NO: 471 - protein, 5 aa, Artificial Sequence
  Synthetic peptide
KNNDG

SEQ ID NO: 472 - protein, 5 aa, Artificial Sequence
  Synthetic peptide
RNNDG

SEQ ID NO: 473 - protein, 7 aa, Artificial Sequence
  Synthetic peptide
NLVGEEY

SEQ ID NO: 474 - protein, 7 aa, Artificial Sequence
  Synthetic peptide
NDSGEIY

SEQ ID NO: 475 - protein, 5 aa, Artificial Sequence
  Synthetic peptide
EPVTG

SEQ ID NO: 476 - protein, 5 aa, Artificial Sequence
  Synthetic peptide
HGMPK

SEQ ID NO: 477 - protein, 5 aa, Artificial Sequence
  Synthetic peptide
HGMAK

SEQ ID NO: 478 - protein, 5 aa, Artificial Sequence
  Synthetic peptide
VPWIF

SEQ ID NO: 479 - protein, 7 aa, Artificial Sequence
  Synthetic peptide
KSSVPFQ

SEQ ID NO: 480 - protein, 7 aa, Artificial Sequence
  Synthetic peptide
KETVNFQ

SEQ ID NO: 481 - protein, 5 aa, Artificial Sequence
  Synthetic peptide
VWSGS

SEQ ID NO: 482 - protein, 5 aa, Artificial Sequence
  Synthetic peptide
IWSGS

SEQ ID NO: 483 - protein, 7 aa, Artificial Sequence
  Synthetic peptide
FSLENWG

SEQ ID NO: 484 - protein, 7 aa, Artificial Sequence
  Synthetic peptide
FSMGRWG

SEQ ID NO: 485 - protein, 7 aa, Artificial Sequence
  Synthetic peptide
FSLVLWG

SEQ ID NO: 486 - protein, 7 aa, Artificial Sequence
  Synthetic peptide
FSLVLWG

SEQ ID NO: 487 - protein, 7 aa, Artificial Sequence
  Synthetic peptide
FSLTNWG

SEQ ID NO: 488 - protein, 5 aa, Artificial Sequence
  Synthetic peptide
PTNQG

SEQ ID NO: 489 - protein, 5 aa, Artificial Sequence
  Synthetic peptide
PTNPG

SEQ ID NO: 490 - protein, 9 aa, Artificial Sequence
  Synthetic peptide
RKLHWNHRT

SEQ ID NO: 491 - protein, 9 aa, Artificial Sequence
  Synthetic peptide
KKYRYRHPT

SEQ ID NO: 492 - protein, 9 aa, Artificial Sequence
  Synthetic peptide
RKAVYQHNT

SEQ ID NO: 493 - protein, 7 aa, Artificial Sequence
  Synthetic peptide
RTLHPRF

SEQ ID NO: 494 - protein, 7 aa, Artificial Sequence
  Synthetic peptide
HFRHPRF

SEQ ID NO: 495 - protein, 7 aa, Artificial Sequence
  Synthetic peptide
RVAHPRF

SEQ ID NO: 496 - protein, 7 aa, Artificial Sequence
  Synthetic peptide
WQAHPRF

SEQ ID NO: 497 - protein, 8 aa, Artificial Sequence
  Synthetic peptide
  misc_feature (5)..(5): Xaa can be any naturally occurring amino acid
  misc_feature (6)..(6): Xaa can be S or A
MKEAXXEK

SEQ ID NO: 498 - protein, 8 aa, Artificial Sequence
  Synthetic peptide
MKEAASEK

SEQ ID NO: 499 - protein, 5 aa, Artificial Sequence
  Synthetic peptide
  MISC_FEATURE (2)..(2): Xaa can be I or V
RXPFG

SEQ ID NO: 500 - protein, 6 aa, Artificial Sequence
  Synthetic peptide
  misc_feature (3)..(3): Xaa can be any naturally occurring amino acid
KGXATP

SEQ ID NO: 501 - protein, 6 aa, Artificial Sequence
  Synthetic peptide
  MISC_FEATURE (2)..(2): Xaa can be M or L
  misc_feature (3)..(3): Xaa can be any naturally occurring amino acid
PXXVGP

SEQ ID NO: 502 - protein, 6 aa, Artificial Sequence
  Synthetic peptide
  misc_feature (3)..(3): Xaa can be any naturally occurring amino acid
  misc_feature (6)..(6): Xaa can be R or Y
PKXDGX

SEQ ID NO: 503 - protein, 6 aa, Artificial Sequence
  Synthetic peptide
  misc_feature (2)..(2): Xaa can be any naturally occurring amino acid
  MISC_FEATURE (6)..(6): Xaa can be E or S
KXDGHX

SEQ ID NO: 504 - protein, 7 aa, Artificial Sequence
  Synthetic peptide
  misc_feature (3)..(3): Xaa can be any naturally occurring amino acid
  MISC_FEATURE (4)..(4): Xaa can be F or Y
  misc_feature (6)..(6): Xaa can be any naturally occurring amino acid
  MISC_FEATURE (7)..(7): Xaa can be R or K
VQXXMXX

SEQ ID NO: 505 - protein, 8 aa, Artificial Sequence
  Synthetic peptide
  misc_feature (3)..(3): Xaa can be any naturally occurring amino acid
  misc_feature (5)..(5): Xaa can be any naturally occurring amino acid
  MISC_FEATURE (6)..(6): Xaa can be G or A
  misc_feature (7)..(7): Xaa can be any naturally occurring amino acid
  MISC_FEATURE (8)..(8): Xaa can be V or A
DRXPXXXX

SEQ ID NO: 506 - protein, 7 aa, Artificial Sequence
  Synthetic peptide
  misc_feature (2)..(2): Xaa can be any naturally occurring amino acid
  misc_feature (5)..(5): Xaa can be any naturally occurring amino acid
  MISC_FEATURE (6)..(6): Xaa can be V or L
DXIDXXW

SEQ ID NO: 507 - protein, 6 aa, Artificial Sequence
  Synthetic peptide
  misc_feature (4)..(4): Xaa can be any naturally occurring amino acid
  MISC_FEATURE (6)..(6): Xaa can be R or Q
RQPXGX

SEQ ID NO: 508 - protein, 6 aa, Artificial Sequence
  Synthetic peptide
  misc_feature (2)..(2): Xaa can be any naturally occurring amino acid
PXHGIH

SEQ ID NO: 509 - protein, 5 aa, Artificial Sequence
  Synthetic peptide
DGDGP

SEQ ID NO: 510 - protein, 8 aa, Artificial Sequence
  Synthetic peptide
  misc_feature (2)..(3): Xaa can be any naturally occurring amino acid
  MISC_FEATURE (4)..(4): Xaa can be N or Q
  misc_feature (7)..(7): Xaa can be any naturally occurring amino acid
  MISC_FEATURE (8)..(8): Xaa can be K or R
HXXXTPXX

SEQ ID NO: 511 - protein, 6 aa, Artificial Sequence
  Synthetic peptide
  MISC_FEATURE (2)..(2): Xaa can be S or A
  misc_feature (3)..(3): Xaa can be any naturally occurring amino acid
  MISC_FEATURE (6)..(6): Xaa can be H or E
KXXNPX

SEQ ID NO: 512 - protein, 6 aa, Artificial Sequence
  Synthetic peptide
  MISC_FEATURE (1)..(1): Xaa can be E, Q, D or N
  misc_feature (2)..(2): Xaa can be any naturally occurring amino acid
XXLPHE

SEQ ID NO: 513 - protein, 5 aa, Artificial Sequence
  Synthetic peptide
  misc_feature (5)..(5): Xaa can be V, I or M
GQYGX

SEQ ID NO: 514 - protein, 6 aa, Artificial Sequence
  Synthetic peptide
  MISC_FEATURE (3)..(3): Xaa can be M or  L
  misc_feature (4)..(4): Xaa can be any naturally occurring amino acid
  MISC_FEATURE (5)..(5): Xaa can be D or N
PRXXXK

SEQ ID NO: 515 - protein, 8 aa, Artificial Sequence
  Synthetic peptide
  MISC_FEATURE (4)..(4): Xaa can be G or Q
  misc_feature (5)..(7): Xaa can be any naturally occurring amino acid
FGQXXXXD

SEQ ID NO: 516 - protein, 7 aa, Artificial Sequence
  Synthetic peptide
  MISC_FEATURE (3)..(3): Xaa can be G, R or S
  MISC_FEATURE (3)..(3): Xaa can be G, R or S
  misc_feature (4)..(4): Xaa can be any naturally occurring amino acid
  misc_feature (6)..(6): Xaa can be any naturally occurring amino acid
DDXXTXK

SEQ ID NO: 517 - protein, 6 aa, Artificial Sequence
  Synthetic peptide
  misc_feature (2)..(2): Xaa can be any naturally occurring amino acid
  MISC_FEATURE (4)..(4): Xaa can be F or P
IXTXDR

SEQ ID NO: 518 - protein, 9 aa, Artificial Sequence
  Synthetic peptide
  misc_feature (2)..(3): Xaa can be any naturally occurring amino acid
  misc_feature (7)..(8): Xaa can be any naturally occurring amino acid
  MISC_FEATURE (9)..(9): Xaa can be F or Y
KXXNIGXXX

SEQ ID NO: 519 - protein, 5 aa, Artificial Sequence
  Synthetic peptide
RVPFG

SEQ ID NO: 520 - protein, 5 aa, Artificial Sequence
  Synthetic peptide
RIPFG

SEQ ID NO: 521 - protein, 5 aa, Artificial Sequence
  Synthetic peptide
RIPFG

SEQ ID NO: 522 - protein, 9 aa, Artificial Sequence
  Synthetic peptide
GGLFRVPFG

SEQ ID NO: 523 - protein, 7 aa, Artificial Sequence
  Synthetic peptide
KGKATPS

SEQ ID NO: 524 - protein, 7 aa, Artificial Sequence
  Synthetic peptide
KGKATPS

SEQ ID NO: 525 - protein, 6 aa, Artificial Sequence
  Synthetic peptide
  MISC_FEATURE (3)..(3): Xaa can be V, S, P, L or R
PLXVGP

SEQ ID NO: 526 - protein, 6 aa, Artificial Sequence
  Synthetic peptide
PKVDGR

SEQ ID NO: 527 - protein, 6 aa, Artificial Sequence
  Synthetic peptide
PKADGR

SEQ ID NO: 528 - protein, 6 aa, Artificial Sequence
  Synthetic peptide
PKADGY

SEQ ID NO: 529 - protein, 6 aa, Artificial Sequence
  Synthetic peptide
PKEDGR

SEQ ID NO: 530 - protein, 6 aa, Artificial Sequence
  Synthetic peptide
PKEDGR

SEQ ID NO: 531 - protein, 6 aa, Artificial Sequence
  Synthetic peptide
KYDGHS

SEQ ID NO: 532 - protein, 6 aa, Artificial Sequence
  Synthetic peptide
KCDGHE

SEQ ID NO: 533 - protein, 7 aa, Artificial Sequence
  Synthetic peptide
VQTFMLR

SEQ ID NO: 534 - protein, 7 aa, Artificial Sequence
  Synthetic peptide
VQIYMAK

SEQ ID NO: 535 - protein, 7 aa, Artificial Sequence
  Synthetic peptide
VQLFMRR

SEQ ID NO: 536 - protein, 7 aa, Artificial Sequence
  Synthetic peptide
VQSYMLR

SEQ ID NO: 537 - protein, 7 aa, Artificial Sequence
  Synthetic peptide
VQLYMDK

SEQ ID NO: 538 - protein, 7 aa, Artificial Sequence
  Synthetic peptide
VQLYMDK

SEQ ID NO: 539 - protein, 7 aa, Artificial Sequence
  Synthetic peptide
DDIDLLW

SEQ ID NO: 540 - protein, 6 aa, Artificial Sequence
  Synthetic peptide
RQPCGQ

SEQ ID NO: 541 - protein, 6 aa, Artificial Sequence
  Synthetic peptide
RQPIGR

SEQ ID NO: 542 - protein, 8 aa, Artificial Sequence
  Synthetic peptide
HPTNTPEK

SEQ ID NO: 543 - protein, 8 aa, Artificial Sequence
  Synthetic peptide
HPVNTPDK

SEQ ID NO: 544 - protein, 8 aa, Artificial Sequence
  Synthetic peptide
HAVQTPSK

SEQ ID NO: 545 - protein, 8 aa, Artificial Sequence
  Synthetic peptide
HTFQTPQR

SEQ ID NO: 546 - protein, 8 aa, Artificial Sequence
  Synthetic peptide
HVNQTPYR

SEQ ID NO: 547 - protein, 8 aa, Artificial Sequence
  Synthetic peptide
HDGNTPAK

SEQ ID NO: 548 - protein, 6 aa, Artificial Sequence
  Synthetic peptide
KSANPE

SEQ ID NO: 549 - protein, 6 aa, Artificial Sequence
  Synthetic peptide
KSINPE

SEQ ID NO: 550 - protein, 6 aa, Artificial Sequence
  Synthetic peptide
KASNPH

SEQ ID NO: 551 - protein, 6 aa, Artificial Sequence
  Synthetic peptide
NALPHE

SEQ ID NO: 552 - protein, 6 aa, Artificial Sequence
  Synthetic peptide
DALPHE

SEQ ID NO: 553 - protein, 6 aa, Artificial Sequence
  Synthetic peptide
EPLPHE

SEQ ID NO: 554 - protein, 6 aa, Artificial Sequence
  Synthetic peptide
EMLPHE

SEQ ID NO: 555 - protein, 6 aa, Artificial Sequence
  Synthetic peptide
QPLPHE

SEQ ID NO: 556 - protein, 5 aa, Artificial Sequence
  Synthetic peptide
GQYGV

SEQ ID NO: 557 - protein, 9 aa, Artificial Sequence
  Synthetic peptide
KIPNIGDKF

SEQ ID NO: 558 - protein, 6 aa, Artificial Sequence
  Synthetic peptide
  MISC_FEATURE (1)..(1): Xaa can be M or L
  MISC_FEATURE (3)..(3): Xaa can be A or S
  MISC_FEATURE (4)..(4): Xaa can be T or A
  misc_feature (5)..(5): Xaa can be any naturally occurring amino acid
XLXXXK

SEQ ID NO: 559 - protein, 9 aa, Artificial Sequence
  Synthetic peptide
  MISC_FEATURE (1)..(1): Xaa can be V or L
  misc_feature (2)..(2): Xaa can be any naturally occurring amino acid
  MISC_FEATURE (3)..(3): Xaa can be A or S
  misc_feature (4)..(4): Xaa can be any naturally occurring amino acid
  misc_feature (7)..(8): Xaa can be any naturally occurring amino acid
XXXXDPXXP

SEQ ID NO: 560 - protein, 7 aa, Artificial Sequence
  Synthetic peptide
  MISC_FEATURE (1)..(1): Xaa can be K or R
  misc_feature (2)..(2): Xaa can be any naturally occurring amino acid
  MISC_FEATURE (3)..(3): Xaa can be I or L
  misc_feature (4)..(4): Xaa can be any naturally occurring amino acid
  MISC_FEATURE (5)..(5): Xaa can be S or T
  MISC_FEATURE (6)..(6): Xaa can be M, L or F
XXXXXXN

SEQ ID NO: 561 - protein, 9 aa, Artificial Sequence
  Synthetic peptide
  MISC_FEATURE (3)..(3): Xaa can be K or R
  misc_feature (5)..(8): Xaa can be any naturally occurring amino acid
TGXMXXXXQ

SEQ ID NO: 562 - protein, 10 aa, Artificial Sequence
  Synthetic peptide
  misc_feature (2)..(2): Xaa can be any naturally occurring amino acid
  MISC_FEATURE (5)..(5): Xaa can be S, T or A
  misc_feature (6)..(9): Xaa can be any naturally occurring amino acid
  MISC_FEATURE (10)..(10): Xaa can be M or L
GXPYXXXXXX

SEQ ID NO: 563 - protein, 6 aa, Artificial Sequence
  Synthetic peptide
  MISC_FEATURE (3)..(3): Xaa can be E, D or A
  misc_feature (4)..(4): Xaa can be any naturally occurring amino acid
  MISC_FEATURE (5)..(5): Xaa can be P or A
WEXXXI

SEQ ID NO: 564 - protein, 9 aa, Artificial Sequence
  Synthetic peptide
  MISC_FEATURE (2)..(2): Xaa can be I or V
  misc_feature (3)..(3): Xaa can be any naturally occurring amino acid
  misc_feature (5)..(6): Xaa can be any naturally occurring amino acid
  misc_feature (8)..(8): Xaa can be any naturally occurring amino acid
EXXHXXFXR

SEQ ID NO: 565 - protein, 8 aa, Artificial Sequence
  Synthetic peptide
  misc_feature (2)..(3): Xaa can be any naturally occurring amino acid
  MISC_FEATURE (4)..(4): Xaa can be T or S
  misc_feature (7)..(7): Xaa can be any naturally occurring amino acid
KXXXHRXK

SEQ ID NO: 566 - protein, 7 aa, Artificial Sequence
  Synthetic peptide
  misc_feature (4)..(4): Xaa can be any naturally occurring amino acid
  misc_feature (6)..(6): Xaa can be any naturally occurring amino acid
TFEXGXK

SEQ ID NO: 567 - protein, 9 aa, Artificial Sequence
  Synthetic peptide
  misc_feature (4)..(4): Xaa can be any naturally occurring amino acid
  MISC_FEATURE (5)..(5): Xaa can be R or A
  misc_feature (6)..(8): Xaa can be any naturally occurring amino acid
  MISC_FEATURE (9)..(9): Xaa can be F or I
WENXXXXXX

SEQ ID NO: 568 - protein, 10 aa, Artificial Sequence
  Synthetic peptide
  MISC_FEATURE (1)..(1): Xaa can be N or T
  MISC_FEATURE (2)..(2): Xaa can be M or F
  misc_feature (4)..(7): Xaa can be any naturally occurring amino acid
  misc_feature (9)..(9): Xaa can be any naturally occurring amino acid
XXFXXXXWXD

SEQ ID NO: 569 - protein, 7 aa, Artificial Sequence
  Synthetic peptide
  MISC_FEATURE (1)..(1): Xaa can be P or A
  MISC_FEATURE (2)..(2): Xaa can be G or A
  MISC_FEATURE (3)..(3): Xaa can be I or V
  MISC_FEATURE (4)..(4): Xaa can be M, I, T or V
  misc_feature (5)..(6): Xaa can be any naturally occurring amino acid
XXXXXXP

SEQ ID NO: 570 - protein, 8 aa, Artificial Sequence
  Synthetic peptide
  misc_feature (2)..(3): Xaa can be any naturally occurring amino acid
  misc_feature (5)..(5): Xaa can be any naturally occurring amino acid
  MISC_FEATURE (7)..(7): Xaa can be Y, W or H
KXXRXSXD

SEQ ID NO: 571 - protein, 9 aa, Artificial Sequence
  Synthetic peptide
  misc_feature (3)..(4): Xaa can be any naturally occurring amino acid
  misc_feature (6)..(7): Xaa can be any naturally occurring amino acid
  MISC_FEATURE (8)..(8): Xaa can be Y or F
  MISC_FEATURE (9)..(9): Xaa can be D or N
EKXXRXXXX

SEQ ID NO: 572 - protein, 7 aa, Artificial Sequence
  Synthetic peptide
  misc_feature (3)..(3): Xaa can be any naturally occurring amino acid
  misc_feature (6)..(6): Xaa can be any naturally occurring amino acid
DTXTPXE

SEQ ID NO: 573 - protein, 5 aa, Artificial Sequence
  Synthetic peptide
  MISC_FEATURE (3)..(3): Xaa can be D or A
WLXQW

SEQ ID NO: 574 - protein, 8 aa, Artificial Sequence
  Synthetic peptide
  MISC_FEATURE (2)..(2): Xaa can be E or N
  misc_feature (3)..(4): Xaa can be any naturally occurring amino acid
  misc_feature (6)..(6): Xaa can be any naturally occurring amino acid
KXXXDXWN

SEQ ID NO: 575 - protein, 5 aa, Artificial Sequence
  Synthetic peptide
  MISC_FEATURE (1)..(1): Xaa can be G or T
XGNGG

SEQ ID NO: 576 - protein, 7 aa, Artificial Sequence
  Synthetic peptide
  MISC_FEATURE (2)..(2): Xaa can be Y,F or W
  misc_feature (4)..(5): Xaa can be any naturally occurring amino acid
  MISC_FEATURE (6)..(6): Xaa can be Q or T
GXDXXXP

SEQ ID NO: 577 - protein, 7 aa, Artificial Sequence
  Synthetic peptide
  MISC_FEATURE (1)..(1): Xaa can be I or V
  misc_feature (3)..(3): Xaa can be any naturally occurring amino acid
  MISC_FEATURE (5)..(5): Xaa can be R or K
  misc_feature (6)..(6): Xaa can be any naturally occurring amino acid
  MISC_FEATURE (7)..(7): Xaa can be C or R
XGXSXXX

SEQ ID NO: 578 - protein, 6 aa, Artificial Sequence
  Synthetic peptide
  MISC_FEATURE (1)..(1): Xaa can be S, A or T
  misc_feature (4)..(4): Xaa can be any naturally occurring amino acid
  MISC_FEATURE (5)..(5): Xaa can be M or L
XTPXXE

SEQ ID NO: 579 - protein, 6 aa, Artificial Sequence
  Synthetic peptide
  MISC_FEATURE (2)..(2): Xaa can be D or Q
  misc_feature (4)..(4): Xaa can be any naturally occurring amino acid
SXWXWE

SEQ ID NO: 580 - protein, 9 aa, Artificial Sequence
  Synthetic peptide
  misc_feature (2)..(3): Xaa can be any naturally occurring amino acid
  MISC_FEATURE (5)..(5): Xaa can be I or T
  misc_feature (6)..(7): Xaa can be any naturally occurring amino acid
  MISC_FEATURE (8)..(8): Xaa can be H or F
DXXYXXXXK

SEQ ID NO: 581 - protein, 8 aa, Artificial Sequence
  Synthetic peptide
  MISC_FEATURE (2)..(2): Xaa can be Y or F
  misc_feature (3)..(5): Xaa can be any naturally occurring amino acid
  MISC_FEATURE (7)..(7): Xaa can be I, V or T
KXXXXLXK

SEQ ID NO: 582 - protein, 6 aa, Artificial Sequence
  Synthetic peptide
  MISC_FEATURE (2)..(2): Xaa can be V or I
  misc_feature (3)..(3): Xaa can be any naturally occurring amino acid
PXXYMQ

SEQ ID NO: 583 - protein, 8 aa, Artificial Sequence
  Synthetic peptide
  misc_feature (5)..(7): Xaa can be any naturally occurring amino acid
  MISC_FEATURE (8)..(8): Xaa can be S or N
WPTGXXXX

SEQ ID NO: 584 - protein, 7 aa, Artificial Sequence
  Synthetic peptide
  misc_feature (2)..(2): Xaa can be any naturally occurring amino acid
  MISC_FEATURE (3)..(3): Xaa can be I or M
  MISC_FEATURE (4)..(4): Xaa can be V or N
  misc_feature (5)..(5): Xaa can be any naturally occurring amino acid
KXXXXWA

SEQ ID NO: 585 - protein, 5 aa, Artificial Sequence
  Synthetic peptide
  MISC_FEATURE (2)..(2): Xaa can be A or P
  MISC_FEATURE (5)..(5): Xaa can be K or R
WXTGX

SEQ ID NO: 586 - protein, 8 aa, Artificial Sequence
  Synthetic peptide
  misc_feature (2)..(3): Xaa can be any naturally occurring amino acid
  MISC_FEATURE (5)..(5): Xaa can be I or V
  misc_feature (6)..(6): Xaa can be any naturally occurring amino acid
  MISC_FEATURE (8)..(8): Xaa can be K or R
YXXLXXPX

SEQ ID NO: 587 - protein, 6 aa, Artificial Sequence
  Synthetic peptide
  MISC_FEATURE (1)..(1): Xaa can be S or A
  misc_feature (3)..(3): Xaa can be any naturally occurring amino acid
  MISC_FEATURE (4)..(4): Xaa can be M or L
XNXXFY

SEQ ID NO: 588 - protein, 6 aa, Artificial Sequence
  Synthetic peptide
  misc_feature (5)..(5): Xaa can be any naturally occurring amino acid
  MISC_FEATURE (6)..(6): Xaa can be I or V
WDGSXX

SEQ ID NO: 589 - protein, 7 aa, Artificial Sequence
  Synthetic peptide
  misc_feature (2)..(3): Xaa can be any naturally occurring amino acid
  MISC_FEATURE (5)..(5): Xaa can be I or V
PXXLXKP

SEQ ID NO: 590 - protein, 6 aa, Artificial Sequence
  Synthetic peptide
  misc_feature (2)..(2): Xaa can be any naturally occurring amino acid
KXDWDG

SEQ ID NO: 591 - protein, 10 aa, Artificial Sequence
  Synthetic peptide
  misc_feature (2)..(5): Xaa can be any naturally occurring amino acid
  misc_feature (7)..(7): Xaa can be any naturally occurring amino acid
  MISC_FEATURE (9)..(9): Xaa can be H or Y
RXXXXKXDXD

SEQ ID NO: 592 - protein, 6 aa, Artificial Sequence
  Synthetic peptide
VDVMGN

SEQ ID NO: 593 - protein, 7 aa, Artificial Sequence
  Synthetic peptide
  misc_feature (2)..(2): Xaa can be any naturally occurring amino acid
  MISC_FEATURE (3)..(3): Xaa can be N or Q
  MISC_FEATURE (4)..(4): Xaa can be Q or N
  misc_feature (5)..(5): Xaa can be any naturally occurring amino acid
EXXXXFY

SEQ ID NO: 594 - protein, 5 aa, Artificial Sequence
  Synthetic peptide
  misc_feature (2)..(2): Xaa can be any naturally occurring amino acid
  MISC_FEATURE (3)..(3): Xaa can be T or S
  MISC_FEATURE (4)..(4): Xaa can be T or S
VXXXN

SEQ ID NO: 595 - protein, 5 aa, Artificial Sequence
  Synthetic peptide
KLHDP

SEQ ID NO: 596 - protein, 7 aa, Artificial Sequence
  Synthetic peptide
  misc_feature (2)..(2): Xaa can be any naturally occurring amino acid
  misc_feature (4)..(4): Xaa can be any naturally occurring amino acid
  MISC_FEATURE (7)..(7): Xaa can be G or N
KXDXDTX

SEQ ID NO: 597 - protein, 6 aa, Artificial Sequence
  Synthetic peptide
  MISC_FEATURE (2)..(2): Xaa can be H or A
  misc_feature (5)..(5): Xaa can be any naturally occurring amino acid
  MISC_FEATURE (6)..(6): Xaa can be S, A or E
YXGWXX

SEQ ID NO: 598 - protein, 5 aa, Artificial Sequence
  Synthetic peptide
  MISC_FEATURE (5)..(5): Xaa can be D, T or E
NPEHX

SEQ ID NO: 599 - protein, 6 aa, Artificial Sequence
  Synthetic peptide
  misc_feature (4)..(4): Xaa can be any naturally occurring amino acid
  MISC_FEATURE (6)..(6): Xaa can be H or R
NPAXQX

SEQ ID NO: 600 - protein, 7 aa, Artificial Sequence
  Synthetic peptide
  MISC_FEATURE (1)..(1): Xaa can be K or R
  misc_feature (5)..(6): Xaa can be any naturally occurring amino acid
  MISC_FEATURE (7)..(7): Xaa can be T or P
XMNKXXX

SEQ ID NO: 601 - protein, 8 aa, Artificial Sequence
  Synthetic peptide
  misc_feature (3)..(5): Xaa can be any naturally occurring amino acid
  MISC_FEATURE (6)..(6): Xaa can be F or Y
  MISC_FEATURE (7)..(7): Xaa can be V or K
DWXXXXXK

SEQ ID NO: 602 - protein, 6 aa, Artificial Sequence
  Synthetic peptide
  MISC_FEATURE (4)..(4): Xaa can be A, P, T or S
  misc_feature (5)..(5): Xaa can be any naturally occurring amino acid
GVNXXK

SEQ ID NO: 603 - protein, 7 aa, Artificial Sequence
  Synthetic peptide
  MISC_FEATURE (1)..(1): Xaa can be I or V
  misc_feature (2)..(2): Xaa can be any naturally occurring amino acid
  MISC_FEATURE (3)..(3): Xaa can be P or R
  misc_feature (6)..(6): Xaa can be any naturally occurring amino acid
XXXEGXK

SEQ ID NO: 604 - protein, 5 aa, Artificial Sequence
  Synthetic peptide
  MISC_FEATURE (4)..(4): Xaa can be S or T
  MISC_FEATURE (5)..(5): Xaa can be M or A
RVFXX

SEQ ID NO: 605 - protein, 8 aa, Artificial Sequence
  Synthetic peptide
  misc_feature (2)..(2): Xaa can be any naturally occurring amino acid
  misc_feature (4)..(5): Xaa can be any naturally occurring amino acid
  MISC_FEATURE (6)..(6): Xaa can be V or I
  MISC_FEATURE (8)..(8): Xaa can be Y or F
NXRXXXWX

SEQ ID NO: 606 - protein, 8 aa, Artificial Sequence
  Synthetic peptide
  misc_feature (2)..(3): Xaa can be any naturally occurring amino acid
  MISC_FEATURE (4)..(4): Xaa can be M, T or L
  misc_feature (5)..(5): Xaa can be any naturally occurring amino acid
YXXXXYNA

SEQ ID NO: 607 - protein, 7 aa, Artificial Sequence
  Synthetic peptide
  misc_feature (2)..(2): Xaa can be any naturally occurring amino acid
  MISC_FEATURE (3)..(3): Xaa can be V or I
  misc_feature (4)..(4): Xaa can be any naturally occurring amino acid
  MISC_FEATURE (5)..(5): Xaa can be N or D
  MISC_FEATURE (6)..(6): Xaa can be I or V
KXXXXXW

SEQ ID NO: 608 - protein, 5 aa, Artificial Sequence
  Synthetic peptide
  MISC_FEATURE (1)..(1): Xaa can be E or D
  MISC_FEATURE (2)..(2): Xaa can be Y or F
  MISC_FEATURE (4)..(4): Xaa can be L or Q
XXQXH

SEQ ID NO: 609 - protein, 6 aa, Artificial Sequence
  Synthetic peptide
  misc_feature (3)..(3): Xaa can be any naturally occurring amino acid
FGXPSI

SEQ ID NO: 610 - protein, 7 aa, Artificial Sequence
  Synthetic peptide
  misc_feature (5)..(6): Xaa can be any naturally occurring amino acid
QLVGXXK

SEQ ID NO: 611 - protein, 8 aa, Artificial Sequence
  Synthetic peptide
  misc_feature (2)..(3): Xaa can be any naturally occurring amino acid
  MISC_FEATURE (5)..(5): Xaa can be I or V
  misc_feature (6)..(6): Xaa can be any naturally occurring amino acid
  MISC_FEATURE (8)..(8): Xaa can be K or R
YXXLXXPX

SEQ ID NO: 612 - protein, 6 aa, Artificial Sequence
  Synthetic peptide
  MISC_FEATURE (2)..(2): Xaa can be Y or K
  misc_feature (4)..(4): Xaa can be any naturally occurring amino acid
  MISC_FEATURE (5)..(5): Xaa can be P or A
WXWXXK

SEQ ID NO: 613 - protein, 7 aa, Artificial Sequence
  Synthetic peptide
  misc_feature (2)..(2): Xaa can be any naturally occurring amino acid
  misc_feature (4)..(4): Xaa can be any naturally occurring amino acid
  MISC_FEATURE (6)..(6): Xaa can be N or K
KXEXHXF

SEQ ID NO: 614 - protein, 9 aa, Artificial Sequence
  Synthetic peptide
  misc_feature (2)..(4): Xaa can be any naturally occurring amino acid
  misc_feature (8)..(8): Xaa can be any naturally occurring amino acid
QXXXWPYXK

SEQ ID NO: 615 - protein, 8 aa, Artificial Sequence
  Synthetic peptide
  misc_feature (2)..(2): Xaa can be any naturally occurring amino acid
  misc_feature (5)..(5): Xaa can be any naturally occurring amino acid
  misc_feature (7)..(7): Xaa can be any naturally occurring amino acid
YXFDXNXR

SEQ ID NO: 616 - protein, 6 aa, Artificial Sequence
  Synthetic peptide
  misc_feature (2)..(2): Xaa can be any naturally occurring amino acid
  MISC_FEATURE (5)..(5): Xaa can be V or I
FXWNXP

SEQ ID NO: 617 - protein, 6 aa, Artificial Sequence
  Synthetic peptide
  MISC_FEATURE (1)..(1): Xaa can be F or W
  MISC_FEATURE (2)..(2): Xaa can be L or M
  misc_feature (4)..(4): Xaa can be any naturally occurring amino acid
XXEXAH

SEQ ID NO: 618 - protein, 6 aa, Artificial Sequence
  Synthetic peptide
  MISC_FEATURE (3)..(3): Xaa can be L or I
  misc_feature (4)..(4): Xaa can be any naturally occurring amino acid
DFXXAT

SEQ ID NO: 619 - protein, 7 aa, Artificial Sequence
  Synthetic peptide
  misc_feature (2)..(2): Xaa can be any naturally occurring amino acid
  misc_feature (5)..(5): Xaa can be any naturally occurring amino acid
KXMSXFV

SEQ ID NO: 620 - protein, 6 aa, Artificial Sequence
  Synthetic peptide
  MISC_FEATURE (2)..(2): Xaa can be Y or K
  misc_feature (4)..(4): Xaa can be any naturally occurring amino acid
  MISC_FEATURE (5)..(5): Xaa can be P or A
WXWXXK

SEQ ID NO: 621 - protein, 7 aa, Artificial Sequence
  Synthetic peptide
  misc_feature (2)..(2): Xaa can be any naturally occurring amino acid
  misc_feature (4)..(4): Xaa can be any naturally occurring amino acid
  MISC_FEATURE (6)..(6): Xaa can be N or K
KXEXHXF

SEQ ID NO: 622 - protein, 9 aa, Artificial Sequence
  Synthetic peptide
  misc_feature (2)..(4): Xaa can be any naturally occurring amino acid
  misc_feature (8)..(8): Xaa can be any naturally occurring amino acid
QXXXWPYXK

SEQ ID NO: 623 - protein, 5 aa, Artificial Sequence
  Synthetic peptide
  MISC_FEATURE (4)..(4): Xaa can be S or F
WPTXT

SEQ ID NO: 624 - protein, 5 aa, Artificial Sequence
  Synthetic peptide
  MISC_FEATURE (3)..(3): Xaa can be T or A
WPXGR

SEQ ID NO: 625 - protein, 6 aa, Artificial Sequence
  Synthetic peptide
  misc_feature (5)..(5): Xaa can be any naturally occurring amino acid
  MISC_FEATURE (6)..(6): Xaa can be G or F
KNWPXX

SEQ ID NO: 626 - protein, 7 aa, Artificial Sequence
  Synthetic peptide
  misc_feature (2)..(3): Xaa can be any naturally occurring amino acid
  MISC_FEATURE (5)..(5): Xaa can be L or I
KXXPXFA

SEQ ID NO: 627 - protein, 6 aa, Artificial Sequence
  Synthetic peptide
  misc_feature (3)..(3): Xaa can be any naturally occurring amino acid
WPXGQV

SEQ ID NO: 628 - protein, 5 aa, Artificial Sequence
  Synthetic peptide
  MISC_FEATURE (1)..(1): Xaa can be V or I
  MISC_FEATURE (2)..(2): Xaa can be L or R
XXKDF

SEQ ID NO: 629 - protein, 5 aa, Artificial Sequence
  Synthetic peptide
  MISC_FEATURE (4)..(4): Xaa can be S or F
WPTXT

SEQ ID NO: 630 - protein, 7 aa, Artificial Sequence
  Synthetic peptide
  misc_feature (2)..(2): Xaa can be any naturally occurring amino acid
  MISC_FEATURE (3)..(3): Xaa can be I or M
  MISC_FEATURE (4)..(4): Xaa can be V or N
  misc_feature (5)..(5): Xaa can be any naturally occurring amino acid
KXXXXWA

SEQ ID NO: 631 - protein, 6 aa, Artificial Sequence
  Sythentic peptide
  MISC_FEATURE (1)..(1): Xaa can be Y or W
  misc_feature (3)..(3): Xaa can be any naturally occurring amino acid
XTXEPF

SEQ ID NO: 632 - protein, 6 aa, Artificial Sequence
  Sythentic peptide
  MISC_FEATURE (1)..(1): Xaa can be A or M
  MISC_FEATURE (2)..(2): Xaa can be P, T or S
  misc_feature (5)..(5): Xaa can be any naturally occurring amino acid
XXWEXF

SEQ ID NO: 633 - protein, 5 aa, Artificial Sequence
  Sythentic peptide
  MISC_FEATURE (2)..(2): Xaa can be P or T
  MISC_FEATURE (3)..(3): Xaa can be R, T or K
  MISC_FEATURE (5)..(5): Xaa can be N or S
RXXFX

SEQ ID NO: 634 - protein, 5 aa, Artificial Sequence
  Sythentic peptide
  MISC_FEATURE (3)..(3): Xaa can be S or A
VYXHW

SEQ ID NO: 635 - protein, 10 aa, Artificial Sequence
  Sythentic peptide
  MISC_FEATURE (1)..(1): Xaa can be W or F
  misc_feature (2)..(3): Xaa can be any naturally occurring amino acid
  misc_feature (6)..(6): Xaa can be any naturally occurring amino acid
  misc_feature (8)..(9): Xaa can be any naturally occurring amino acid
XXXKPXWXXM

SEQ ID NO: 636 - protein, 7 aa, Artificial Sequence
  Sythentic peptide
  misc_feature (3)..(3): Xaa can be any naturally occurring amino acid
  MISC_FEATURE (4)..(4): Xaa can be S or A
  misc_feature (6)..(6): Xaa can be any naturally occurring amino acid
KGXXHXF

SEQ ID NO: 637 - protein, 7 aa, Artificial Sequence
  Sythentic peptide
  misc_feature (3)..(3): Xaa can be any naturally occurring amino acid
  misc_feature (5)..(5): Xaa can be any naturally occurring amino acid
  MISC_FEATURE (7)..(7): Xaa can be A or S
KGXVXFX

SEQ ID NO: 638 - protein, 7 aa, Artificial Sequence
  Sythentic peptide
  MISC_FEATURE (1)..(1): Xaa can be I or V
  misc_feature (2)..(2): Xaa can be any naturally occurring amino acid
  misc_feature (4)..(4): Xaa can be any naturally occurring amino acid
XXHXTID

SEQ ID NO: 639 - protein, 7 aa, Artificial Sequence
  Sythentic peptide
  misc_feature (4)..(5): Xaa can be any naturally occurring amino acid
MLSXXVN

SEQ ID NO: 640 - protein, 8 aa, Artificial Sequence
  Sythentic peptide
  misc_feature (2)..(2): Xaa can be any naturally occurring amino acid
  misc_feature (5)..(6): Xaa can be any naturally occurring amino acid
KXYSXXVR

SEQ ID NO: 641 - protein, 6 aa, Artificial Sequence
  Synthetic peptide
  misc_feature (2)..(2): Xaa can be any naturally occurring amino acid
  MISC_FEATURE (3)..(3): Xaa can be V or K
KXXVNP

SEQ ID NO: 642 - protein, 5 aa, Artificial Sequence
  Synthetic peptide
  MISC_FEATURE (1)..(1): Xaa can be R, K or H
XEPGD

SEQ ID NO: 643 - protein, 9 aa, Artificial Sequence
  Synthetic peptide
  misc_feature (2)..(3): Xaa can be any naturally occurring amino acid
  misc_feature (5)..(5): Xaa can be any naturally occurring amino acid
  misc_feature (8)..(8): Xaa can be any naturally occurring amino acid
CXXIXNEXC

SEQ ID NO: 644 - protein, 5 aa, Artificial Sequence
  Synthetic peptide
  MISC_FEATURE (4)..(4): Xaa can be S or N
ESRXI

SEQ ID NO: 645 - protein, 6 aa, Artificial Sequence
  Synthetic peptide
  misc_feature (4)..(4): Xaa can be any naturally occurring amino acid
  MISC_FEATURE (5)..(5): Xaa can be Q or N
HPDXXL

SEQ ID NO: 646 - protein, 6 aa, Artificial Sequence
  Synthetic peptide
  misc_feature (3)..(3): Xaa can be any naturally occurring amino acid
  MISC_FEATURE (5)..(5): Xaa can be F or Y
  MISC_FEATURE (6)..(6): Xaa can be E or D
RYXHXX

SEQ ID NO: 647 - protein, 7 aa, Artificial Sequence
  Synthetic peptide
  MISC_FEATURE (2)..(2): Xaa can be A or S
  misc_feature (3)..(3): Xaa can be any naturally occurring amino acid
  misc_feature (6)..(6): Xaa can be any naturally occurring amino acid
FXXRQXP

SEQ ID NO: 648 - protein, 5 aa, Artificial Sequence
  Synthetic peptide
  MISC_FEATURE (3)..(3): Xaa can be A or P
QDXRN

SEQ ID NO: 649 - protein, 7 aa, Artificial Sequence
  Synthetic peptide
  misc_feature (2)..(3): Xaa can be any naturally occurring amino acid
  MISC_FEATURE (4)..(4): Xaa can be I, L or M
LXXXNQQ

SEQ ID NO: 650 - protein, 6 aa, Artificial Sequence
  Synthetic peptide
  MISC_FEATURE (1)..(1): Xaa can be V or A
  misc_feature (2)..(2): Xaa can be any naturally occurring amino acid
  MISC_FEATURE (6)..(6): Xaa can be W or F
XXDGAX

SEQ ID NO: 651 - protein, 6 aa, Artificial Sequence
  Synthetic peptide
  misc_feature (2)..(2): Xaa can be any naturally occurring amino acid
  MISC_FEATURE (6)..(6): Xaa can be M, T or S
CXLPEX

SEQ ID NO: 652 - protein, 7 aa, Artificial Sequence
  Synthetic peptide
  misc_feature (2)..(3): Xaa can be any naturally occurring amino acid
  MISC_FEATURE (6)..(6): Xaa can be T, H or S
FXXMQXK

SEQ ID NO: 653 - protein, 6 aa, Artificial Sequence
  Synthetic peptide
  MISC_FEATURE (3)..(3): Xaa can be G, A or S
  misc_feature (4)..(4): Xaa can be any naturally occurring amino acid
GHXXLR

SEQ ID NO: 654 - protein, 9 aa, Artificial Sequence
  Synthetic peptide
  misc_feature (2)..(3): Xaa can be any naturally occurring amino acid
  MISC_FEATURE (4)..(4): Xaa can be D or E
  misc_feature (6)..(7): Xaa can be any naturally occurring amino acid
  MISC_FEATURE (9)..(9): Xaa can be V or E
WXXXYXXLX

SEQ ID NO: 655 - protein, 5 aa, Artificial Sequence
  Synthetic peptide
  MISC_FEATURE (2)..(2): Xaa can be H, N or D
  MISC_FEATURE (3)..(3): Xaa can be Y or F
FXXPR

SEQ ID NO: 656 - protein, 5 aa, Artificial Sequence
  Synthetic peptide
  MISC_FEATURE (3)..(3): Xaa can be F or Y
PEXTS

SEQ ID NO: 657 - protein, 9 aa, Artificial Sequence
  Synthetic peptide
  misc_feature (3)..(3): Xaa can be any naturally occurring amino acid
  misc_feature (6)..(8): Xaa can be any naturally occurring amino acid
CDXPSXXXC

SEQ ID NO: 658 - protein, 8 aa, Artificial Sequence
  Synthetic peptide
  MISC_FEATURE (1)..(1): Xaa can be F or Y
  misc_feature (2)..(3): Xaa can be any naturally occurring amino acid
  misc_feature (7)..(7): Xaa can be any naturally occurring amino acid
XXXNGHXF

SEQ ID NO: 659 - protein, 9 aa, Artificial Sequence
  Synthetic peptide
  misc_feature (2)..(2): Xaa can be any naturally occurring amino acid
  misc_feature (5)..(5): Xaa can be any naturally occurring amino acid
  misc_feature (7)..(8): Xaa can be any naturally occurring amino acid
YXICXEXXC

SEQ ID NO: 660 - protein, 7 aa, Artificial Sequence
  Synthetic peptide
  misc_feature (5)..(6): Xaa can be any naturally occurring amino acid
DCMGXXC

SEQ ID NO: 661 - protein, 7 aa, Artificial Sequence
  Synthetic peptide
  MISC_FEATURE (1)..(1): Xaa can be M or L
  misc_feature (2)..(2): Xaa can be any naturally occurring amino acid
  misc_feature (6)..(6): Xaa can be any naturally occurring amino acid
  MISC_FEATURE (7)..(7): Xaa can be D or E
XXTGLXX

SEQ ID NO: 662 - protein, 6 aa, Artificial Sequence
  Synthetic peptide
  misc_feature (2)..(2): Xaa can be any naturally occurring amino acid
MXLGYY

SEQ ID NO: 663 - protein, 6 aa, Artificial Sequence
  Synthetic peptide
  MISC_FEATURE (3)..(3): Xaa can be L or T
  misc_feature (5)..(5): Xaa can be any naturally occurring amino acid
  MISC_FEATURE (6)..(6): Xaa can be Y or H
MPXGXX

SEQ ID NO: 664 - protein, 6 aa, Artificial Sequence
  Synthetic peptide
  MISC_FEATURE (1)..(1): Xaa can be F or L
  misc_feature (5)..(5): Xaa can be any naturally occurring amino acid
  MISC_FEATURE (6)..(6): Xaa can be I or L
XQTGXX

SEQ ID NO: 665 - protein, 6 aa, Artificial Sequence
  Synthetic peptide
  misc_feature (2)..(2): Xaa can be any naturally occurring amino acid
  MISC_FEATURE (3)..(3): Xaa can be T or S
KXXCPC

SEQ ID NO: 666 - protein, 5 aa, Artificial Sequence
  Synthetic peptide
  MISC_FEATURE (4)..(4): Xaa can be T, S or D
CKDXC

SEQ ID NO: 667 - protein, 5 aa, Artificial Sequence
  Synthetic peptide
  MISC_FEATURE (3)..(3): Xaa can be V or A
  MISC_FEATURE (5)..(5): Xaa can be E or Q
CGXFX

SEQ ID NO: 668 - protein, 8 aa, Artificial Sequence
  Synthetic peptide
  misc_feature (3)..(3): Xaa can be any naturally occurring amino acid
  MISC_FEATURE (4)..(4): Xaa can be I, V, A or E
  misc_feature (6)..(7): Xaa can be any naturally occurring amino acid
  MISC_FEATURE (8)..(8): Xaa can be I, M or L
SNXXAXXX

SEQ ID NO: 669 - protein, 8 aa, Artificial Sequence
  Synthetic peptide
  misc_feature (3)..(3): Xaa can be any naturally occurring amino acid
  misc_feature (5)..(5): Xaa can be any naturally occurring amino acid
  misc_feature (7)..(7): Xaa can be any naturally occurring amino acid
  MISC_FEATURE (8)..(8): Xaa can be K or R
PTXLXHXX

SEQ ID NO: 670 - protein, 5 aa, Artificial Sequence
  Synthetic peptide
WPVNN

SEQ ID NO: 671 - protein, 9 aa, Artificial Sequence
  Synthetic peptide
  MISC_FEATURE (1)..(1): Xaa can be V, I or A
  MISC_FEATURE (4)..(4): Xaa can be G or D
  misc_feature (5)..(8): Xaa can be any naturally occurring amino acid
XCNXXXXXC

SEQ ID NO: 672 - protein, 5 aa, Artificial Sequence
  Synthetic peptide
  MISC_FEATURE (1)..(1): Xaa can be K or R
  MISC_FEATURE (4)..(4): Xaa can be Y or S
XNPXL

SEQ ID NO: 673 - protein, 10 aa, Artificial Sequence
  Synthetic peptide
  misc_feature (2)..(4): Xaa can be any naturally occurring amino acid
  misc_feature (7)..(7): Xaa can be any naturally occurring amino acid
  misc_feature (9)..(9): Xaa can be any naturally occurring amino acid
CXXXPMXVXC

SEQ ID NO: 674 - protein, 7 aa, Artificial Sequence
  Synthetic peptide
  MISC_FEATURE (2)..(2): Xaa can be L or M
  MISC_FEATURE (3)..(3): Xaa can be K, Q or T
  misc_feature (5)..(6): Xaa can be any naturally occurring amino acid
GXXFXXD

SEQ ID NO: 675 - protein, 6 aa, Artificial Sequence
  Synthetic peptide
  MISC_FEATURE (1)..(1): Xaa can be I or A
  misc_feature (4)..(4): Xaa can be any naturally occurring amino acid
  MISC_FEATURE (5)..(5): Xaa can be P, A or K
XPMXXN

SEQ ID NO: 676 - protein, 10 aa, Artificial Sequence
  Synthetic peptide
  misc_feature (2)..(2): Xaa can be any naturally occurring amino acid
  misc_feature (5)..(5): Xaa can be any naturally occurring amino acid
  MISC_FEATURE (6)..(6): Xaa can be H or T
  misc_feature (7)..(9): Xaa can be any naturally occurring amino acid
WXWCXXXXXC

SEQ ID NO: 677 - protein, 7 aa, Artificial Sequence
  Synthetic peptide
  misc_feature (2)..(3): Xaa can be any naturally occurring amino acid
  MISC_FEATURE (5)..(5): Xaa can be Q, M, H or E
  MISC_FEATURE (6)..(6): Xaa can be T or H
FXXMXXK

SEQ ID NO: 678 - protein, 8 aa, Artificial Sequence
  Synthetic peptide
  misc_feature (2)..(2): Xaa can be any naturally occurring amino acid
  misc_feature (4)..(4): Xaa can be any naturally occurring amino acid
  MISC_FEATURE (5)..(5): Xaa can be V or I
  misc_feature (6)..(6): Xaa can be any naturally occurring amino acid
KXEXXXWR

SEQ ID NO: 679 - protein, 6 aa, Artificial Sequence
  Synthetic peptide
  MISC_FEATURE (3)..(3): Xaa can be N or T
  misc_feature (5)..(5): Xaa can be any naturally occurring amino acid
CHXGXC

SEQ ID NO: 680 - protein, 5 aa, Artificial Sequence
  Synthetic peptide
HEPGD

SEQ ID NO: 681 - protein, 5 aa, Artificial Sequence
  Synthetic peptide
REPGD

SEQ ID NO: 682 - protein, 5 aa, Artificial Sequence
  Synthetic peptide
KEPGD

SEQ ID NO: 683 - protein, 5 aa, Artificial Sequence
  Synthetic peptide
REPGD

SEQ ID NO: 684 - protein, 9 aa, Artificial Sequence
  Synthetic peptide
CKKIVNETC

SEQ ID NO: 685 - protein, 5 aa, Artificial Sequence
  Synthetic peptide
ESRSI

SEQ ID NO: 686 - protein, 5 aa, Artificial Sequence
  Synthetic peptide
ESRNI

SEQ ID NO: 687 - protein, 6 aa, Artificial Sequence
  Synthetic peptide
HPDVNL

SEQ ID NO: 688 - protein, 6 aa, Artificial Sequence
  Synthetic peptide
HPDGNL

SEQ ID NO: 689 - protein, 6 aa, Artificial Sequence
  Synthetic peptide
HPDKNL

SEQ ID NO: 690 - protein, 6 aa, Artificial Sequence
  Synthetic peptide
HPDEQL

SEQ ID NO: 691 - protein, 6 aa, Artificial Sequence
  Synthetic peptide
HPDTQL

SEQ ID NO: 692 - protein, 6 aa, Artificial Sequence
  Synthetic peptide
RYCHFD

SEQ ID NO: 693 - protein, 6 aa, Artificial Sequence
  Synthetic peptide
RYYHYD

SEQ ID NO: 694 - protein, 6 aa, Artificial Sequence
  Synthetic peptide
RYKHFD

SEQ ID NO: 695 - protein, 7 aa, Artificial Sequence
  Synthetic peptide
FSFRQQP

SEQ ID NO: 696 - protein, 7 aa, Artificial Sequence
  Synthetic peptide
FAHRQQP

SEQ ID NO: 697 - protein, 7 aa, Artificial Sequence
  Synthetic peptide
FAHRQRP

SEQ ID NO: 698 - protein, 7 aa, Artificial Sequence
  Synthetic peptide
FATRQGP

SEQ ID NO: 699 - protein, 5 aa, Artificial Sequence
  Synthetic peptide
QDPRN

SEQ ID NO: 700 - protein, 7 aa, Artificial Sequence
  Synthetic peptide
LLQLNQQ

SEQ ID NO: 701 - protein, 7 aa, Artificial Sequence
  Synthetic peptide
LSLMNQQ

SEQ ID NO: 702 - protein, 7 aa, Artificial Sequence
  Synthetic peptide
LFWINQQ

SEQ ID NO: 703 - protein, 7 aa, Artificial Sequence
  Synthetic peptide
LQKLNQQ

SEQ ID NO: 704 - protein, 7 aa, Artificial Sequence
  Synthetic peptide
LILLNQQ

SEQ ID NO: 705 - protein, 6 aa, Artificial Sequence
  Synthetic peptide
APDGAF

SEQ ID NO: 706 - protein, 6 aa, Artificial Sequence
  Synthetic peptide
VQDGAF

SEQ ID NO: 707 - protein, 6 aa, Artificial Sequence
  Synthetic peptide
ACDGAF

SEQ ID NO: 708 - protein, 6 aa, Artificial Sequence
  Synthetic peptide
AIDGAF

SEQ ID NO: 709 - protein, 6 aa, Artificial Sequence
  Synthetic peptide
AIDGAF

SEQ ID NO: 710 - protein, 6 aa, Artificial Sequence
  Synthetic peptide
CSLPES

SEQ ID NO: 711 - protein, 6 aa, Artificial Sequence
  Synthetic peptide
CPLPET

SEQ ID NO: 712 - protein, 6 aa, Artificial Sequence
  Synthetic peptide
CVLPES

SEQ ID NO: 713 - protein, 6 aa, Artificial Sequence
  Synthetic peptide
CRLPET

SEQ ID NO: 714 - protein, 6 aa, Artificial Sequence
  Synthetic peptide
CPLPET

SEQ ID NO: 715 - protein, 6 aa, Artificial Sequence
  Synthetic peptide
CDLPET

SEQ ID NO: 716 - protein, 7 aa, Artificial Sequence
  Synthetic peptide
FKKMQSK

SEQ ID NO: 717 - protein, 7 aa, Artificial Sequence
  Synthetic peptide
FLFMQHK

SEQ ID NO: 718 - protein, 6 aa, Artificial Sequence
  Synthetic peptide
GHSTLR

SEQ ID NO: 719 - protein, 6 aa, Artificial Sequence
  Synthetic peptide
GHSALR

SEQ ID NO: 720 - protein, 6 aa, Artificial Sequence
  Synthetic peptide
GHGTLR

SEQ ID NO: 721 - protein, 6 aa, Artificial Sequence
  Synthetic peptide
GHGRLR

SEQ ID NO: 722 - protein, 6 aa, Artificial Sequence
  Synthetic peptide
GHGFLR

SEQ ID NO: 723 - protein, 9 aa, Artificial Sequence
  Synthetic peptide
WQIDYTSLV

SEQ ID NO: 724 - protein, 5 aa, Artificial Sequence
  Synthetic peptide
FDFPR

SEQ ID NO: 725 - protein, 5 aa, Artificial Sequence
  Synthetic peptide
FDYPR

SEQ ID NO: 726 - protein, 5 aa, Artificial Sequence
  Synthetic peptide
FNYPR

SEQ ID NO: 727 - protein, 5 aa, Artificial Sequence
  Synthetic peptide
PEFTS

SEQ ID NO: 728 - protein, 8 aa, Artificial Sequence
  Synthetic peptide
YYQNGHEF

SEQ ID NO: 729 - protein, 8 aa, Artificial Sequence
  Synthetic peptide
YHVNGHRF

SEQ ID NO: 730 - protein, 7 aa, Artificial Sequence
  Synthetic peptide
LITGLPD

SEQ ID NO: 731 - protein, 7 aa, Artificial Sequence
  Synthetic peptide
MYTGLPE

SEQ ID NO: 732 - protein, 7 aa, Artificial Sequence
  Synthetic peptide
LWTGLEE

SEQ ID NO: 733 - protein, 7 aa, Artificial Sequence
  Synthetic peptide
LLTGLAD

SEQ ID NO: 734 - protein, 7 aa, Artificial Sequence
  Synthetic peptide
LLTGLLD

SEQ ID NO: 735 - protein, 7 aa, Artificial Sequence
  Synthetic peptide
MDTGLVD

SEQ ID NO: 736 - protein, 6 aa, Artificial Sequence
  Synthetic peptide
MRLGYY

SEQ ID NO: 737 - protein, 6 aa, Artificial Sequence
  Synthetic peptide
MPTGGH

SEQ ID NO: 738 - protein, 6 aa, Artificial Sequence
  Synthetic peptide
LQTGTL

SEQ ID NO: 739 - protein, 6 aa, Artificial Sequence
  Synthetic peptide
LQTGKL

SEQ ID NO: 740 - protein, 6 aa, Artificial Sequence
  Synthetic peptide
FQTGDI

SEQ ID NO: 741 - protein, 5 aa, Artificial Sequence
  Synthetic peptide
CGAFE

SEQ ID NO: 742 - protein, 5 aa, Artificial Sequence
  Synthetic peptide
CGVFQ

SEQ ID NO: 743 - protein, 8 aa, Artificial Sequence
  Synthetic peptide
SNRVASFL

SEQ ID NO: 744 - protein, 8 aa, Artificial Sequence
  Synthetic peptide
SNKAARQM

SEQ ID NO: 745 - protein, 8 aa, Artificial Sequence
  Synthetic peptide
SNSAAVDL

SEQ ID NO: 746 - protein, 8 aa, Artificial Sequence
  Synthetic peptide
SNDVAKII

SEQ ID NO: 747 - protein, 8 aa, Artificial Sequence
  Synthetic peptide
SNAVAQVL

SEQ ID NO: 748 - protein, 8 aa, Artificial Sequence
  Synthetic peptide
SNNVAFEI

SEQ ID NO: 749 - protein, 8 aa, Artificial Sequence
  Synthetic peptide
PTGLDHHR

SEQ ID NO: 750 - protein, 8 aa, Artificial Sequence
  Synthetic peptide
PTYLIHER

SEQ ID NO: 751 - protein, 9 aa, Artificial Sequence
  Synthetic peptide
ICNDSSRRC

SEQ ID NO: 752 - protein, 9 aa, Artificial Sequence
  Synthetic peptide
ACNGHSITC

SEQ ID NO: 753 - protein, 9 aa, Artificial Sequence
  Synthetic peptide
VCNGHADTC

SEQ ID NO: 754 - protein, 9 aa, Artificial Sequence
  Synthetic peptide
ACNGEHSQC

SEQ ID NO: 755 - protein, 5 aa, Artificial Sequence
  Synthetic peptide
RNPSL

SEQ ID NO: 756 - protein, 5 aa, Artificial Sequence
  Synthetic peptide
KNPSL

SEQ ID NO: 757 - protein, 7 aa, Artificial Sequence
  Synthetic peptide
GLTFQAD

SEQ ID NO: 758 - protein, 7 aa, Artificial Sequence
  Synthetic peptide
GLQFAFD

SEQ ID NO: 759 - protein, 7 aa, Artificial Sequence
  Synthetic peptide
GMKFTRD

SEQ ID NO: 760 - protein, 7 aa, Artificial Sequence
  Synthetic peptide
GLQFPSD

SEQ ID NO: 761 - protein, 7 aa, Artificial Sequence
  Synthetic peptide
GLKFSPD

SEQ ID NO: 762 - protein, 7 aa, Artificial Sequence
  Synthetic peptide
GLTFTPD

SEQ ID NO: 763 - protein, 6 aa, Artificial Sequence
  Synthetic peptide
APMDAN

SEQ ID NO: 764 - protein, 6 aa, Artificial Sequence
  Synthetic peptide
IPMDPN

SEQ ID NO: 765 - protein, 6 aa, Artificial Sequence
  Synthetic peptide
APMPKN

SEQ ID NO: 766 - protein, 6 aa, Artificial Sequence
  Synthetic peptide
APMFKN

SEQ ID NO: 767 - protein, 7 aa, Artificial Sequence
  Synthetic peptide
FLFMQHK

SEQ ID NO: 768 - protein, 7 aa, Artificial Sequence
  Synthetic peptide
FFDMETK

SEQ ID NO: 769 - protein, 7 aa, Artificial Sequence
  Synthetic peptide
FEEMQTK

SEQ ID NO: 770 - protein, 6 aa, Artificial Sequence
  Synthetic peptide
CHTGPC

SEQ ID NO: 771 - protein, 7 aa, Artificial Sequence
  Synthetic peptide
  MISC_FEATURE (1)..(1): Xaa can be V or I
  misc_feature (5)..(5): Xaa can be any naturally occurring amino acid
  MISC_FEATURE (7)..(7): Xaa can be S or A
XPEFXGX

SEQ ID NO: 772 - protein, 7 aa, Artificial Sequence
  Synthetic peptide
  MISC_FEATURE (2)..(2): Xaa can be I, V or M
  misc_feature (4)..(5): Xaa can be any naturally occurring amino acid
  MISC_FEATURE (6)..(6): Xaa can be L or M
YXDXXXN

SEQ ID NO: 773 - protein, 5 aa, Artificial Sequence
  Synthetic peptide
DDKGK

SEQ ID NO: 774 - protein, 6 aa, Artificial Sequence
  Synthetic peptide
  misc_feature (2)..(2): Xaa can be any naturally occurring amino acid
KXPEEP

SEQ ID NO: 775 - protein, 6 aa, Artificial Sequence
  Synthetic peptide
  MISC_FEATURE (1)..(1): Xaa can be L or M
  misc_feature (2)..(2): Xaa can be any naturally occurring amino acid
XXLPDK

SEQ ID NO: 776 - protein, 6 aa, Artificial Sequence
  Synthetic peptide
  MISC_FEATURE (1)..(1): Xaa can be I, V or Y
  misc_feature (3)..(4): Xaa can be any naturally occurring amino acid
XDXXGN

SEQ ID NO: 777 - protein, 6 aa, Artificial Sequence
  Synthetic peptide
  MISC_FEATURE (2)..(2): Xaa can be V or I
  MISC_FEATURE (3)..(3): Xaa can be V or I
  MISC_FEATURE (4)..(4): Xaa can be V or I
EXXXDK

SEQ ID NO: 778 - protein, 6 aa, Artificial Sequence
  Synthetic peptide
  MISC_FEATURE (1)..(1): Xaa can be M or L
  MISC_FEATURE (2)..(2): Xaa can be W or Y
XXWMDK

SEQ ID NO: 779 - protein, 4 aa, Artificial Sequence
  Synthetic peptide
NPVE

SEQ ID NO: 780 - protein, 6 aa, Artificial Sequence
  Synthetic peptide
  misc_feature (4)..(5): Xaa can be any naturally occurring amino acid
CMNXXC

SEQ ID NO: 781 - protein, 6 aa, Artificial Sequence
  Synthetic peptide
  MISC_FEATURE (1)..(1): Xaa can be R or K
  misc_feature (3)..(3): Xaa can be any naturally occurring amino acid
  MISC_FEATURE (4)..(4): Xaa can be M or L
XDXXGR

SEQ ID NO: 782 - protein, 8 aa, Artificial Sequence
  Synthetic peptide
  MISC_FEATURE (1)..(1): Xaa can be I or V
  misc_feature (2)..(3): Xaa can be any naturally occurring amino acid
  misc_feature (5)..(5): Xaa can be any naturally occurring amino acid
  MISC_FEATURE (7)..(7): Xaa can be D or E
XXXPXYXK

SEQ ID NO: 783 - protein, 7 aa, Artificial Sequence
  Synthetic peptide
  misc_feature (2)..(2): Xaa can be any naturally occurring amino acid
  MISC_FEATURE (4)..(4): Xaa can be T or V
  misc_feature (6)..(6): Xaa can be any naturally occurring amino acid
PXGXLXK

SEQ ID NO: 784 - protein, 8 aa, Artificial Sequence
  Synthetic peptide
  MISC_FEATURE (1)..(1): Xaa can be V or I
  misc_feature (2)..(3): Xaa can be any naturally occurring amino acid
  misc_feature (6)..(6): Xaa can be any naturally occurring amino acid
XXXQPXKP

SEQ ID NO: 785 - protein, 5 aa, Artificial Sequence
  Synthetic peptide
  misc_feature (3)..(3): Xaa can be any naturally occurring amino acid
  MISC_FEATURE (5)..(5): Xaa can be R or K
DTXPX

SEQ ID NO: 786 - protein, 10 aa, Artificial Sequence
  Synthetic peptide
  misc_feature (2)..(3): Xaa can be any naturally occurring amino acid
  misc_feature (6)..(7): Xaa can be any naturally occurring amino acid
  misc_feature (9)..(9): Xaa can be any naturally occurring amino acid
CXXPWXXEXC

SEQ ID NO: 787 - protein, 7 aa, Artificial Sequence
  Synthetic peptide
  MISC_FEATURE (2)..(2): Xaa can be W or F
  misc_feature (3)..(3): Xaa can be any naturally occurring amino acid
  MISC_FEATURE (4)..(4): Xaa can be Q, I or V
WXXXPDK

SEQ ID NO: 788 - protein, 4 aa, Artificial Sequence
  Synthetic peptide
PPWW

SEQ ID NO: 789 - protein, 4 aa, Artificial Sequence
  Synthetic peptide
  MISC_FEATURE (1)..(1): Xaa can be L or I
  MISC_FEATURE (3)..(3): Xaa can be K or R
XNXP

SEQ ID NO: 790 - protein, 8 aa, Artificial Sequence
  Synthetic peptide
  MISC_FEATURE (2)..(2): Xaa can be I or L
  misc_feature (3)..(3): Xaa can be any naturally occurring amino acid
  misc_feature (5)..(5): Xaa can be any naturally occurring amino acid
  MISC_FEATURE (6)..(6): Xaa can be H or P
  misc_feature (7)..(7): Xaa can be any naturally occurring amino acid
PXXNXXXW

SEQ ID NO: 791 - protein, 7 aa, Artificial Sequence
  Synthetic peptide
  MISC_FEATURE (1)..(1): Xaa can be F or Y
  misc_feature (2)..(2): Xaa can be any naturally occurring amino acid
  misc_feature (4)..(5): Xaa can be any naturally occurring amino acid
  MISC_FEATURE (6)..(6): Xaa can be L, I or M
XXHXXXN

SEQ ID NO: 792 - protein, 8 aa, Artificial Sequence
  Synthetic peptide
  MISC_FEATURE (1)..(1): Xaa can be P or W
  misc_feature (3)..(4): Xaa can be any naturally occurring amino acid
  MISC_FEATURE (6)..(6): Xaa can be D or N
XFXXMXKP

SEQ ID NO: 793 - protein, 5 aa, Artificial Sequence
  Synthetic peptide
  MISC_FEATURE (2)..(2): Xaa can be F, Y or W
KXTHP

SEQ ID NO: 794 - protein, 7 aa, Artificial Sequence
  Synthetic peptide
  misc_feature (2)..(2): Xaa can be any naturally occurring amino acid
  misc_feature (5)..(6): Xaa can be any naturally occurring amino acid
  MISC_FEATURE (7)..(7): Xaa can be W or Y
YXPTXXX

SEQ ID NO: 795 - protein, 8 aa, Artificial Sequence
  Synthetic peptide
  misc_feature (2)..(2): Xaa can be any naturally occurring amino acid
  misc_feature (5)..(5): Xaa can be any naturally occurring amino acid
  MISC_FEATURE (7)..(7): Xaa can be L, M or I
  MISC_FEATURE (8)..(8): Xaa can be L, V or I
PXAIXDXX

SEQ ID NO: 796 - protein, 7 aa, Artificial Sequence
  Synthetic peptide
  misc_feature (2)..(2): Xaa can be any naturally occurring amino acid
  misc_feature (4)..(5): Xaa can be any naturally occurring amino acid
  MISC_FEATURE (6)..(6): Xaa can be L or M
YXDXXXN

SEQ ID NO: 797 - protein, 6 aa, Artificial Sequence
  Synthetic peptide
  MISC_FEATURE (2)..(2): Xaa can be W or N
  misc_feature (3)..(3): Xaa can be any naturally occurring amino acid
  MISC_FEATURE (4)..(4): Xaa can be W or R
  MISC_FEATURE (4)..(4): Xaa can be W or R
  misc_feature (5)..(5): Xaa can be any naturally occurring amino acid
CXXXXC

SEQ ID NO: 798 - protein, 8 aa, Artificial Sequence
  Synthetic peptide
  misc_feature (2)..(2): Xaa can be any naturally occurring amino acid
  misc_feature (6)..(7): Xaa can be any naturally occurring amino acid
KXDPDXXW

SEQ ID NO: 799 - protein, 6 aa, Artificial Sequence
  Synthetic peptide
  MISC_FEATURE (1)..(1): Xaa can be R or K
  MISC_FEATURE (3)..(3): Xaa can be Y or F
  MISC_FEATURE (4)..(4): Xaa can be L, I, V or M
  MISC_FEATURE (6)..(6): Xaa can be E or D
XCXXCX

SEQ ID NO: 800 - protein, 5 aa, Artificial Sequence
  Synthetic peptide
  MISC_FEATURE (5)..(5): Xaa can be D or E
WCWKX

SEQ ID NO: 801 - protein, 6 aa, Artificial Sequence
  Synthetic peptide
  MISC_FEATURE (1)..(1): Xaa can be V or I
  misc_feature (2)..(2): Xaa can be any naturally occurring amino acid
  MISC_FEATURE (3)..(3): Xaa can be L, F or M
XXXPHW

SEQ ID NO: 802 - protein, 7 aa, Artificial Sequence
  Synthetic peptide
  misc_feature (2)..(2): Xaa can be any naturally occurring amino acid
  MISC_FEATURE (4)..(4): Xaa can be S or T
  misc_feature (5)..(6): Xaa can be any naturally occurring amino acid
PXLXXXE

SEQ ID NO: 803 - protein, 9 aa, Artificial Sequence
  Synthetic peptide
  misc_feature (2)..(2): Xaa can be any naturally occurring amino acid
  MISC_FEATURE (3)..(3): Xaa can be I or V
  misc_feature (4)..(4): Xaa can be any naturally occurring amino acid
  misc_feature (6)..(7): Xaa can be any naturally occurring amino acid
  MISC_FEATURE (9)..(9): Xaa can be F or W
PXXXEXXMX

SEQ ID NO: 804 - protein, 7 aa, Artificial Sequence
  Synthetic peptide
  misc_feature (5)..(6): Xaa can be any naturally occurring amino acid
  MISC_FEATURE (7)..(7): Xaa can be W or F
DPYQXXX

SEQ ID NO: 805 - protein, 8 aa, Artificial Sequence
  Synthetic peptide
  MISC_FEATURE (1)..(1): Xaa can be V or I
  misc_feature (3)..(3): Xaa can be any naturally occurring amino acid
  misc_feature (5)..(7): Xaa can be any naturally occurring amino acid
XPXLXXXE

SEQ ID NO: 806 - protein, 4 aa, Artificial Sequence
  Synthetic peptide
YNPF

SEQ ID NO: 807 - protein, 6 aa, Artificial Sequence
  Synthetic peptide
  misc_feature (3)..(3): Xaa can be any naturally occurring amino acid
  MISC_FEATURE (5)..(5): Xaa can be N or D
PVXFXK

SEQ ID NO: 808 - protein, 6 aa, Artificial Sequence
  Synthetic peptide
  misc_feature (2)..(3): Xaa can be any naturally occurring amino acid
PXXFYN

SEQ ID NO: 809 - protein, 6 aa, Artificial Sequence
  Synthetic peptide
  misc_feature (3)..(4): Xaa can be any naturally occurring amino acid
PYXXYQ

SEQ ID NO: 810 - protein, 5 aa, Artificial Sequence
  Synthetic peptide
  MISC_FEATURE (1)..(1): Xaa can be R or H
  MISC_FEATURE (2)..(2): Xaa can be R or K
  MISC_FEATURE (3)..(3): Xaa can be P or W
XXXFF

SEQ ID NO: 811 - protein, 6 aa, Artificial Sequence
  Synthetic peptide
  misc_feature (2)..(2): Xaa can be any naturally occurring amino acid
  misc_feature (5)..(5): Xaa can be any naturally occurring amino acid
KXRPXW

SEQ ID NO: 812 - protein, 8 aa, Artificial Sequence
  Synthetic peptide
  misc_feature (2)..(2): Xaa can be any naturally occurring amino acid
  misc_feature (5)..(7): Xaa can be any naturally occurring amino acid
CXNWXXXC

SEQ ID NO: 813 - protein, 7 aa, Artificial Sequence
  Synthetic peptide
  MISC_FEATURE (2)..(2): Xaa can be I, W, M or L
  misc_feature (4)..(5): Xaa can be any naturally occurring amino acid
CXNXXDC

SEQ ID NO: 814 - protein, 7 aa, Artificial Sequence
  Synthetic peptide
  misc_feature (2)..(2): Xaa can be any naturally occurring amino acid
  misc_feature (4)..(4): Xaa can be any naturally occurring amino acid
  misc_feature (6)..(6): Xaa can be any naturally occurring amino acid
KXDXMXN

SEQ ID NO: 815 - protein, 8 aa, Artificial Sequence
  Synthetic peptide
  misc_feature (2)..(2): Xaa can be any naturally occurring amino acid
  misc_feature (4)..(5): Xaa can be any naturally occurring amino acid
  misc_feature (7)..(7): Xaa can be any naturally occurring amino acid
WXKXXGXW

SEQ ID NO: 816 - protein, 7 aa, Artificial Sequence
  Synthetic peptide
  misc_feature (2)..(2): Xaa can be any naturally occurring amino acid
  MISC_FEATURE (5)..(5): Xaa can be S or A
PXDTXPR

SEQ ID NO: 817 - protein, 6 aa, Artificial Sequence
  Synthetic peptide
  MISC_FEATURE (4)..(4): Xaa can be Y, F or W
  MISC_FEATURE (5)..(5): Xaa can be L or M
PPTXXG

SEQ ID NO: 818 - protein, 7 aa, Artificial Sequence
  Synthetic peptide
  MISC_FEATURE (1)..(1): Xaa can be Y or F
  misc_feature (2)..(2): Xaa can be any naturally occurring amino acid
  MISC_FEATURE (3)..(3): Xaa can be Y or F
  misc_feature (4)..(5): Xaa can be any naturally occurring amino acid
XXXXXFN

SEQ ID NO: 819 - protein, 9 aa, Artificial Sequence
  Synthetic peptide
  MISC_FEATURE (1)..(1): Xaa can be L or M
  misc_feature (2)..(3): Xaa can be any naturally occurring amino acid
  misc_feature (7)..(7): Xaa can be any naturally occurring amino acid
XXXGWNXKP

SEQ ID NO: 820 - protein, 7 aa, Artificial Sequence
  Synthetic peptide
  misc_feature (2)..(2): Xaa can be any naturally occurring amino acid
  MISC_FEATURE (3)..(3): Xaa can be I, V or F
  misc_feature (5)..(5): Xaa can be any naturally occurring amino acid
KXXPXYL

SEQ ID NO: 821 - protein, 7 aa, Artificial Sequence
  Synthetic peptide
  misc_feature (2)..(3): Xaa can be any naturally occurring amino acid
  MISC_FEATURE (4)..(4): Xaa can be I or V
  MISC_FEATURE (7)..(7): Xaa can be M or L
YXXXPWX

SEQ ID NO: 822 - protein, 5 aa, Artificial Sequence
  Synthetic peptide
GAGGG

SEQ ID NO: 823 - protein, 8 aa, Artificial Sequence
  Synthetic peptide
  misc_feature (2)..(2): Xaa can be any naturally occurring amino acid
  MISC_FEATURE (3)..(3): Xaa can be N or D
  misc_feature (4)..(4): Xaa can be any naturally occurring amino acid
  misc_feature (6)..(7): Xaa can be any naturally occurring amino acid
CXXXPXXC

SEQ ID NO: 824 - protein, 6 aa, Artificial Sequence
  Synthetic peptide
  misc_feature (2)..(2): Xaa can be any naturally occurring amino acid
  MISC_FEATURE (4)..(4): Xaa can be M or L
  MISC_FEATURE (5)..(5): Xaa can be F, M or  Y
HXPXXY

SEQ ID NO: 825 - protein, 6 aa, Artificial Sequence
  Synthetic peptide
  MISC_FEATURE (5)..(5): Xaa can be S or G
PDDIXK

SEQ ID NO: 826 - protein, 7 aa, Artificial Sequence
  Synthetic peptide
  misc_feature (3)..(4): Xaa can be any naturally occurring amino acid
FPXXWYP

SEQ ID NO: 827 - protein, 5 aa, Artificial Sequence
  Synthetic peptide
  misc_feature (4)..(4): Xaa can be any naturally occurring amino acid
DMNXH

SEQ ID NO: 828 - protein, 7 aa, Artificial Sequence
  Synthetic peptide
  MISC_FEATURE (1)..(1): Xaa can be K or R
  MISC_FEATURE (2)..(2): Xaa can be L, M or I
  misc_feature (4)..(4): Xaa can be any naturally occurring amino acid
  MISC_FEATURE (7)..(7): Xaa can be S or N
XXVXQSX

SEQ ID NO: 829 - protein, 6 aa, Artificial Sequence
  Synthetic peptide
  misc_feature (3)..(4): Xaa can be any naturally occurring amino acid
WDXXDG

SEQ ID NO: 830 - protein, 8 aa, Artificial Sequence
  Synthetic peptide
  misc_feature (2)..(3): Xaa can be any naturally occurring amino acid
  misc_feature (5)..(6): Xaa can be any naturally occurring amino acid
  MISC_FEATURE (7)..(7): Xaa can be L or I
  MISC_FEATURE (8)..(8): Xaa can be T or S
PXXNXXXX

SEQ ID NO: 831 - protein, 6 aa, Artificial Sequence
  Synthetic peptide
  MISC_FEATURE (1)..(1): Xaa can be V, M or I
  misc_feature (5)..(5): Xaa can be any naturally occurring amino acid
XVPEXK

SEQ ID NO: 832 - protein, 8 aa, Artificial Sequence
  Synthetic peptide
  misc_feature (2)..(2): Xaa can be any naturally occurring amino acid
  MISC_FEATURE (3)..(3): Xaa can be V or I
  MISC_FEATURE (4)..(4): Xaa can be F, Y or W
  misc_feature (5)..(5): Xaa can be any naturally occurring amino acid
  misc_feature (7)..(7): Xaa can be any naturally occurring amino acid
PXXXXNXP

SEQ ID NO: 833 - protein, 5 aa, Artificial Sequence
  Synthetic peptide
  MISC_FEATURE (4)..(4): Xaa can be K or R
  MISC_FEATURE (5)..(5): Xaa can be H or Y
SGPXX

SEQ ID NO: 834 - protein, 6 aa, Artificial Sequence
  Synthetic peptide
  misc_feature (2)..(3): Xaa can be any naturally occurring amino acid
KXXFPQ

SEQ ID NO: 835 - protein, 7 aa, Artificial Sequence
  Synthetic peptide
  misc_feature (3)..(4): Xaa can be any naturally occurring amino acid
  misc_feature (6)..(6): Xaa can be any naturally occurring amino acid
PDXXWXK

SEQ ID NO: 836 - protein, 5 aa, Artificial Sequence
  Synthetic peptide
  MISC_FEATURE (3)..(3): Xaa can be L or M
  MISC_FEATURE (4)..(4): Xaa can be F or M
QPXXY

SEQ ID NO: 837 - protein, 7 aa, Artificial Sequence
  Synthetic peptide
  MISC_FEATURE (1)..(1): Xaa can be Y or F
  misc_feature (2)..(2): Xaa can be any naturally occurring amino acid
  MISC_FEATURE (5)..(5): Xaa can be F, Y or M
XXCTXMC

SEQ ID NO: 838 - protein, 8 aa, Artificial Sequence
  Synthetic peptide
  MISC_FEATURE (1)..(1): Xaa can be F or W
  misc_feature (2)..(2): Xaa can be any naturally occurring amino acid
  misc_feature (4)..(5): Xaa can be any naturally occurring amino acid
  MISC_FEATURE (6)..(6): Xaa can be L, M or I
  MISC_FEATURE (7)..(7): Xaa can be Q or N
  MISC_FEATURE (8)..(8): Xaa can be R or K
XXPXXXXX

SEQ ID NO: 839 - protein, 6 aa, Artificial Sequence
  Synthetic peptide
  MISC_FEATURE (1)..(1): Xaa can be I or V
  misc_feature (5)..(5): Xaa can be any naturally occurring amino acid
  MISC_FEATURE (6)..(6): Xaa can be P or C
XCWSXX

SEQ ID NO: 840 - protein, 6 aa, Artificial Sequence
  Synthetic peptide
  misc_feature (3)..(3): Xaa can be any naturally occurring amino acid
  MISC_FEATURE (5)..(5): Xaa can be V or I
PDXPXS

SEQ ID NO: 841 - protein, 7 aa, Artificial Sequence
  Synthetic peptide
  MISC_FEATURE (2)..(2): Xaa can be L or I
  misc_feature (3)..(3): Xaa can be any naturally occurring amino acid
  misc_feature (5)..(5): Xaa can be any naturally occurring amino acid
PXXGXPW

SEQ ID NO: 842 - protein, 6 aa, Artificial Sequence
  Synthetic peptide
  misc_feature (5)..(5): Xaa can be any naturally occurring amino acid
  MISC_FEATURE (6)..(6): Xaa can be Y, M or L
ELPRXX

SEQ ID NO: 843 - protein, 6 aa, Artificial Sequence
  Synthetic peptide
  MISC_FEATURE (6)..(6): Xaa can be D or W
PESHNX

SEQ ID NO: 844 - protein, 7 aa, Artificial Sequence
  Synthetic peptide
  misc_feature (2)..(3): Xaa can be any naturally occurring amino acid
  misc_feature (6)..(6): Xaa can be any naturally occurring amino acid
  MISC_FEATURE (7)..(7): Xaa can be Y or W
YXXTLXX

SEQ ID NO: 845 - protein, 6 aa, Artificial Sequence
  Synthetic peptide
  MISC_FEATURE (1)..(1): Xaa can be V or I
  misc_feature (2)..(2): Xaa can be any naturally occurring amino acid
  misc_feature (5)..(5): Xaa can be any naturally occurring amino acid
XXWNXP

SEQ ID NO: 846 - protein, 7 aa, Artificial Sequence
  Synthetic peptide
  MISC_FEATURE (2)..(2): Xaa can be W, Y or F
  misc_feature (4)..(5): Xaa can be any naturally occurring amino acid
  MISC_FEATURE (7)..(7): Xaa can be G or P
GXDXXDX

SEQ ID NO: 847 - protein, 7 aa, Artificial Sequence
  Synthetic peptide
  misc_feature (2)..(2): Xaa can be any naturally occurring amino acid
  MISC_FEATURE (3)..(3): Xaa can be T,S or N
  MISC_FEATURE (7)..(7): Xaa can be E or D
KXXHPGX

SEQ ID NO: 848 - protein, 5 aa, Artificial Sequence
  Synthetic peptide
  misc_feature (3)..(3): Xaa can be any naturally occurring amino acid
MMXHI

SEQ ID NO: 849 - protein, 7 aa, Artificial Sequence
  Synthetic peptide
  misc_feature (3)..(3): Xaa can be any naturally occurring amino acid
  misc_feature (6)..(6): Xaa can be any naturally occurring amino acid
  MISC_FEATURE (7)..(7): Xaa can be K or R
KPXLGXX

SEQ ID NO: 850 - protein, 5 aa, Artificial Sequence
  Synthetic peptide
  MISC_FEATURE (2)..(2): Xaa can be S or D
NXSMN

SEQ ID NO: 851 - protein, 5 aa, Artificial Sequence
  Synthetic peptide
  misc_feature (2)..(3): Xaa can be any naturally occurring amino acid
WXXWF

SEQ ID NO: 852 - protein, 6 aa, Artificial Sequence
  Synthetic peptide
  misc_feature (4)..(4): Xaa can be any naturally occurring amino acid
GELXGQ

SEQ ID NO: 853 - protein, 6 aa, Artificial Sequence
  Synthetic peptide
  MISC_FEATURE (1)..(1): Xaa can be M, L or F
  misc_feature (2)..(2): Xaa can be any naturally occurring amino acid
XXNPQQ

SEQ ID NO: 854 - protein, 6 aa, Artificial Sequence
  Synthetic peptide
  misc_feature (5)..(5): Xaa can be any naturally occurring amino acid
TTESXV

SEQ ID NO: 855 - protein, 5 aa, Artificial Sequence
  Synthetic peptide
  MISC_FEATURE (4)..(4): Xaa can be G or A
KDVXE

SEQ ID NO: 856 - protein, 8 aa, Artificial Sequence
  Synthetic peptide
  misc_feature (3)..(3): Xaa can be any naturally occurring amino acid
  MISC_FEATURE (5)..(5): Xaa can be F, W or M
  misc_feature (7)..(7): Xaa can be any naturally occurring amino acid
KPXDXGXK

SEQ ID NO: 857 - protein, 6 aa, Artificial Sequence
  Synthetic peptide
  misc_feature (2)..(2): Xaa can be any naturally occurring amino acid
VXADGT

SEQ ID NO: 858 - protein, 5 aa, Artificial Sequence
  Synthetic peptide
  MISC_FEATURE (2)..(2): Xaa can be A or P
  MISC_FEATURE (3)..(3): Xaa can be A or T
MXXAD

SEQ ID NO: 859 - protein, 6 aa, Artificial Sequence
  Synthetic peptide
  misc_feature (3)..(3): Xaa can be any naturally occurring amino acid
  MISC_FEATURE (6)..(6): Xaa can be D or G
VPXPKX

SEQ ID NO: 860 - protein, 6 aa, Artificial Sequence
  Synthetic peptide
  misc_feature (2)..(2): Xaa can be any naturally occurring amino acid
  MISC_FEATURE (5)..(5): Xaa can be T or S
QXKPXD

SEQ ID NO: 861 - protein, 6 aa, Artificial Sequence
  Synthetic peptide
  MISC_FEATURE (2)..(2): Xaa can be T or S
  misc_feature (3)..(3): Xaa can be any naturally occurring amino acid
FXXDGF

SEQ ID NO: 862 - protein, 6 aa, Artificial Sequence
  Synthetic peptide
  misc_feature (2)..(2): Xaa can be any naturally occurring amino acid
  MISC_FEATURE (3)..(3): Xaa can be R or K
  MISC_FEATURE (6)..(6): Xaa can be V or A
WXXVYX

SEQ ID NO: 863 - protein, 8 aa, Artificial Sequence
  Synthetic peptide
  MISC_FEATURE (1)..(1): Xaa can be C or S
  MISC_FEATURE (3)..(3): Xaa can be T or S
  misc_feature (5)..(7): Xaa can be any naturally occurring amino acid
  MISC_FEATURE (8)..(8): Xaa can be Y or F
XTXEXXXX

SEQ ID NO: 864 - protein, 6 aa, Artificial Sequence
  Synthetic peptide
  misc_feature (2)..(2): Xaa can be any naturally occurring amino acid
  MISC_FEATURE (6)..(6): Xaa can be T or I
YXETCX

SEQ ID NO: 865 - protein, 7 aa, Artificial Sequence
  Synthetic peptide
VQHYMHR

SEQ ID NO: 866 - protein, 6 aa, Artificial Sequence
  Synthetic peptide
RQPQGR

SEQ ID NO: 867 - protein, 7 aa, Artificial Sequence
  Synthetic peptide
DCMGTFC

SEQ ID NO: 868 - protein, 8 aa, Artificial Sequence
  Synthetic peptide
KREIVFWR

SEQ ID NO: 869 - protein, 7 aa, Artificial Sequence
  Synthetic peptide
  misc_feature (3)..(3): Xaa can be any naturally occurring amino acid
  misc_feature (6)..(6): Xaa can be any naturally occurring amino acid
PDXGVXP

SEQ ID NO: 870 - DNA, 53 bp, Artificial Sequence
  Synthetic
  misc_feature (34)..(38): n is a, c, g, or t
tcgtcggcagcgtcagatgtgtataagagacagnnnnnccagtctggccaggg

SEQ ID NO: 871 - DNA, 54 bp, Artificial Sequence
  Synthetic
ccagtactacggcatcactgctgtctcttatacacatctccgagcccacgagac